European Patent Specification EP 4 382 599 B1, published April 8, 2026. Title: Probiotic compositions and uses thereof. Applicant: The University of British Columbia. Application EP EP24157215.5, filed February 12, 2024. The sequence listing filed with the application follows.

SEQUENCE LISTING (75 sequences)

SEQ ID NO: 1 - DNA, 21 bp, synthetic construct
  misc_feature 1..21: note = Primer
  source 1..21: mol_type = other DNA
gagctcgaattctcatgtttg

SEQ ID NO: 2 - DNA, 21 bp, synthetic construct
  misc_feature 1..21: note = Primer
  source 1..21: mol_type = other DNA
ggatcctctagagtcgacctg

SEQ ID NO: 3 - DNA, 52 bp, synthetic construct
  misc_feature 1..52: note = Primer
  source 1..52: mol_type = other DNA
gcatgcctgcaggtcgactctagaggatccgttatatacgctcgatttttgc

SEQ ID NO: 4 - DNA, 51 bp, synthetic construct
  misc_feature 1..51: note = Primer
  source 1..51: mol_type = other DNA
ataagctgtcaaacatgagaattcgagctcttattcatggctcatacgttg

SEQ ID NO: 5 - DNA, 20 bp, synthetic construct
  misc_feature 1..20: note = Primer
  source 1..20: mol_type = other DNA
cgttatggactgcaacatgg

SEQ ID NO: 6 - DNA, 20 bp, synthetic construct
  misc_feature 1..20: note = Primer
  source 1..20: mol_type = other DNA
gcaaacggcctaaatacagc

SEQ ID NO: 7 - DNA, 60 bp, synthetic construct
  misc_feature 1..60: note = Primer
  source 1..60: mol_type = other DNA
tgccaagcttgcatgcctgcaggtcgactctagaggatccattccggggatccgtcgacc

SEQ ID NO: 8 - DNA, 60 bp, synthetic construct
  misc_feature 1..60: note = Primer
  source 1..60: mol_type = other DNA
ctgatcagtgataagctgtcaaacatgagaattcgagctctgtaggctggagctgcttcg

SEQ ID NO: 9 - DNA, 60 bp, synthetic construct
  misc_feature 1..60: note = Primer
  source 1..60: mol_type = other DNA
ccaattactaccagcttcagcactaccagcactaccaatcctctttcggtaataaatctt

SEQ ID NO: 10 - DNA, 60 bp, synthetic construct
  misc_feature 1..60: note = Primer
  source 1..60: mol_type = other DNA
gtgagcgcgcgtaatacgactcactatagggcggatccggtctatcctttatgggagaac

SEQ ID NO: 11 - DNA, 90 bp, synthetic construct
  misc_feature 1..90: note = Primer
  source 1..90: mol_type = other DNA
gtgctgaagctggtagtaattggagtcatccacaatttgaaaaaggtagtgctggtagtgctgctggtagtcacggttacgtatcggcag

SEQ ID NO: 12 - DNA, 60 bp, synthetic construct
  misc_feature 1..60: note = Primer
  source 1..60: mol_type = other DNA
aattcaccactaccagcagcactaccagcactaccaccgtcaaacttaacgtcaataacg

SEQ ID NO: 13 - DNA, 60 bp, synthetic construct
  misc_feature 1..60: note = Primer
  source 1..60: mol_type = other DNA
agtgctggtagtgctgctggtagtggtgaatttaaagttacctatagtggtagtgacagc

SEQ ID NO: 14 - DNA, 60 bp, synthetic construct
  misc_feature 1..60: note = Primer
  source 1..60: mol_type = other DNA
cgatatcaagcttatcgataccgtcgacctcgagaattcccgtcaagataatccgataag

SEQ ID NO: 15 - DNA, 28 bp, synthetic construct
  misc_feature 1..28: note = Primer
  source 1..28: mol_type = other DNA
gaattgggtaccgggccccccctcgagg

SEQ ID NO: 16 - DNA, 28 bp, synthetic construct
  misc_feature 1..28: note = Primer
  source 1..28: mol_type = other DNA
gccctatagtgagtcgtattacgcgcgc

SEQ ID NO: 17 - DNA, 22 bp, synthetic construct
  misc_feature 1..22: note = Primer
  source 1..22: mol_type = other DNA
aactgttggggttacttcggta

SEQ ID NO: 18 - DNA, 21 bp, synthetic construct
  misc_feature 1..21: note = Primer
  source 1..21: mol_type = other DNA
ctggttgttgctcaggtgttt

SEQ ID NO: 19 - protein, 485 aa, Vibrio cholerae
MKKQPKMTAIALILSGISGLAYGHGYVSAVENGVAEGRVTLCKFAANGTGEKNTHCGAIQYEPQSVEGPDGFPVTGPRDGKIASAESALAAALDEQTADRWVKRPIQAGPQTFEWTFTANHVTKDWKYYITKPNWNPNQPLSRDAFDLNPFCVVEGNMVQPPKRVSHECIVPEREGYQVILAVWDVGDTAASFYNVIDVKFDGNGPVLPDWNPAGQIIPSMDLSIGDTVYTRVFDNDGENPAYRTELKIDSETLTKANQWSYALATKINQTQKQQRAGQLNGDQFVPVYGTNPIYLKEGSGLKSVEIGYQIEAPQPEYSLTVSGLAKEYEIGEQPIQLDLTLEAQGEMSAELTVYNHHQKPLASWSQAMTDGELKSITLELSEAKAGHHMLVSRIKDRDGNLQDQQTLDFMLVEPQTPPTPGDYDFVFPNGLKEYVAGTKVLASDGAIYQCKPWPYSGYCQQWTSNATQYQPGTGSHWEMAWDKR

SEQ ID NO: 20 - protein, 180 aa, Vibrio cholerae
HGYVSAVENGVAEGRVTLCKFAANGTGEKNTHCGAIQYEPQSVEGPDGFPVTGPRDGKIASAESALAAALDEQTADRWVKRPIQAGPQTFEWTFTANHVTKDWKYYITKPNWNPNQPLSRDAFDLNPFCVVEGNMVQPPKRVSHECIVPEREGYQVILAVWDVGDTAASFYNVIDVKFDG

SEQ ID NO: 21 - protein, 1229 aa, Lactobacillus reuteri
MYLGGLIMLSRKNYKETIRKQTPTKQYYTIKKLTVGVTSVLIGLSFMGELEGDSVHADTMTASSESTSVTSTTAQDGLKKSPQLYLQVTDTNNPSTPLSASSTGTSKNVTSSAAVQVKSASDEEDSDSTLAKGENKFARSAVKDSVTDGKTSTAEINPAKLSSPALITQLNQSLAKSSTSDAAKANDELEIKATDPTNYPNCGDVYGPLFELDASGQLVNKDEVISLKDMYIFQILKLVNTKDSDFQYVILTMNRKDTADRSVYLFVTGSNYSNAVVVKVKPNDTYELSKTGYSVTYTEPTTINGHYVDGTFYVTGSTYDDGFIMPDWQLQHLQIIYSLGNYDPSNTDATSVCEIMPSYEKVPVIKYSGVPSNISQPKVYITGFTGQEFNVTDIINNYKKVFKGYYLQNPNVASMGTLSQFENGGYYLKTYYDNDGNVDFKGLYHQIDDQGTMSVSVLNADNKTIVGPENILAGKSHNFNFNGHNWIARNPYVTSSAHEVILKYAKLGSVIPVDENGNKINDGWQYVNDPDDASKATSPYEKAPVIDGYVAVNPDETIVLPHNLSSDTKIYYRKRIKVTYSGSDSKTYDGNPANFEPTTVQWSGLKGLNTSTLTSADFTWNTADKKAPTDAGKYTLSLNTTGEAALRKANPNYDLKTISGSYTYTINPLGIDKVTYSGSDSKTYDGNPANFEPTTVQWSGLKGLNTSTLTSADFTWNTADKKAPTDAGKYTLSLNTTGEAALRKANPNYDLKTISGSYTYTINPLGIDKVTYSGSDSKTYDGNPANFEPTTVQWSGLKGLNTSTLTSADFTWNTADKKAPTDAGKYTLSLNTTGEAALRKANPNYDLKTISGSYTYTINPLGIDKVTYSGSDSKTYDGNPANFEPTTVQWSGLKGLNTSTLTSADFTWNTADKKAPTDAGKYTLSLNTTGEAALRKANPNYDLKTISGSYTYTINPLGIDKVTYSGSDSKTYDGNPANFEPTTVQWSGLKGLNTSTLTSADFTWNTADKKAPTDAGKYTLSLNTTGEAALRKANPNYDLKTISGSYTYTINPLGIVTVNYKGYDKKVYDGQPGTINPGKLTWSKLPDGTSLKMPTWSIDDFAWETADGLAPTAVGTYRIILTDAGKAALKKINPNYDLSSITGVFTYEIKPAQTPEILGQTPEQQPGQNTNQSGAENGFGSSTRPNASTNSNLNQLPQTGNEHSNTALAGLALAFLTAMLGLGKKRKHD

SEQ ID NO: 22 - DNA, 540 bp, synthetic construct
  misc_feature 1..540: note = Harmonized Sequence
  source 1..540: mol_type = other DNA
cacggttacgtatcggcagttgaaaacggtgtagccgaagggcgtgtaactctttgtaaatttgcagccaacggtacaggggagaaaaacacacactgtggtgcaattcaatatgaacctcaatctgtagaaggtcctgatggtttccctgtaacaggtcctcgtgatggtaaaattgcctctgcagaatctgcccttgcagccgcacttgatgaacaaactgcagaccgttgggtcaagcgtcctattcaagcaggtcctcaaactttcgagtggaccttcactgcaaaccacgtaacgaaggattggaagtactacattactaagccaaactggaacccaaaccagcctcttagccgtgatgcatttgacttgaaccctttctgtgtcgtagaagggaacatggttcagcctcctaagcgtgtatctcacgaatgtattgttcctgaacgtgaagggtaccaggtaatcctagcagtctgggatgtaggtgatactgcagcctcgttctacaacgttattgacgttaagtttgacggt

SEQ ID NO: 23 - DNA, 3690 bp, Lactobacillus reuteri
  source 1..3690: mol_type = genomic DNA
ttgtatttaggagggttaataatgctatcaagaaaaaattataaggaaactatacgaaaacagacacctacaaaacagtactatactattaagaaattaactgttggggttacttcggtattaattggtctatcctttatgggagaactagaaggggatagcgttcatgcggacacgatgacagcaagcagtgagtcaacaagtgttacgtcgacgactgctcaggatggtttaaaaaaatctccacaactctatttgcaagttactgatacaaataacccaagtacaccattaagtgcttcatccacagggactagtaagaatgttacctcatcagctgcggtacaagtgaagtccgctagtgatgaagaagatagtgattctacactagctaagggagaaaataaatttgctcggtcagcagtaaaagattcagtcactgatgggaaaacaagtacagcagaaattaatccggcaaaattaagcagtcctgctttaataacgcaactcaaccaatccttagctaagagcagtacgagtgatgcagcaaaagctaatgatgagttagaaattaaagcaacagatccgactaattatccaaactgtggcgatgtgtatgggccattatttgaattggatgctagcggacagcttgttaataaagatgaagttatatctcttaaagatatgtatattttccaaatattgaaattagtaaatacaaaagatagtgactttcaatatgtaatattaacaatgaatcgtaaagatactgcagataggtctgtatatctttttgtaactggaagcaattatagtaatgctgttgttgttaaagtaaagccaaatgatacttatgaattaagtaaaactggatatagtgttacttatacagaaccaacaactataaatggacattatgttgatggaactttttatgttacaggaagtacttacgatgatggttttataatgccagattggcaactgcagcaccttcagattatatatagtttaggaaattatgatccaagcaatactgacgcaacatcagtttgtgaaataatgccaagttatgaaaaggtaccggtaattaaatatagtggagtaccttcaaatattagccaacctaaggtttacattaccgggtttacgggtcaagagtttaacgttacagatattattaacaattataagaaagtttttaagggctactatcttcaaaatcctaatgtggcgtccatgggaactctttcccaatttgagaatggtggttattacttaaagacatattatgataatgatggtaatgttgactttaagggcttgtatcatcaaattgatgatcagggaacaatgagtgtgagtgttcttaatgcagataataaaacaattgttggacctgaaaatattcttgctggtaaatcgcataactttaactttaatggtcataactggattgcgcggaatccttatgtcactagttcagctcacgaagtcatattaaagtatgctaagttaggttcagttattcctgttgatgaaaacggaaataaaataaacgatggatggcaatatgttaatgatccagatgatgcttccaaagccactagcccatatgaaaaagcgccagttatcgatggttatgtagctgtaaatccagatgaaacgatcgttcttcctcataacttaagtagtgacacaaagatttattaccgaaagaggattaaagttacctatagtggtagtgacagcaagacctacgatggtaacccagctaacttcgagccaacgacagttcagtggagtggcttgaaaggactgaacacttcaaccttaacgtccgctgacttcacgtggaatactgcggataagaaggcaccaacggatgccggtaagtacacacttagtttgaatacgaccggagaagcagccttacgtaaggctaacccgaactatgatctcaagacaattagcggtagttacacctacacgattaatccactagggattgataaagttacctatagtggtagtgacagcaagacctacgatggtaacccagctaacttcgagccaacgacagttcagtggagtggcttgaaaggactgaacacttcaaccttaacgtccgctgacttcacgtggaatactgcggataagaaggcaccaacggatgccggtaagtacacacttagtttgaatacgaccggagaagcagccttacgtaaggctaacccgaactatgatctcaagacaattagcggtagttacacctacacgattaatccactagggattgataaagttacctatagtggtagtgacagcaagacctacgatggtaacccagctaacttcgagccaacgacagttcagtggagtggcttgaaaggactgaacacttcaaccttaacgtccgctgacttcacgtggaatactgcggataagaaggcaccaacggatgccggtaagtacacacttagtttgaatacgaccggagaagcagccttacgtaaggctaacccgaactatgatctcaagacaattagcggtagttacacctacacgattaatccactagggattgataaagttacctatagtggtagtgacagcaagacctacgatggtaacccagctaacttcgagccaacgacagttcagtggagtggcttgaaaggactgaacacttcaaccttaacgtccgctgacttcacgtggaatactgcggataagaaggcaccaacggatgccggtaagtacacacttagtttgaatacgaccggagaagcagccttacgtaaggctaacccgaactatgatctcaagacaattagcggtagttacacctacacgattaatccactagggattgataaagttacctatagtggtagtgacagcaagacctacgatggtaacccagctaacttcgagccaacgacagttcagtggagtggcttgaaaggactgaacacttcaaccttaacgtccgctgacttcacgtggaatactgcggataagaaggcaccaacggatgccggtaagtacacacttagtttgaatacgaccggagaagcagccttacgtaaggctaacccgaactatgatctcaagacaattagcggtagttacacctacacgattaatccactagggattgtgactgtaaattacaagggctatgataagaaagtctatgatggtcaacctggaacgattaatccgggtaaattaacgtggagtaagttgccagatggtacttcattgaagatgccaacatggagtatagatgatttcgcttgggaaacagctgatggcttagcaccaacggcagtaggaacttatcggattatcttgacggatgctggtaaggctgcactaaagaagattaatccaaattatgacttaagcagtattactggtgtctttacttatgaaattaagccagcacagacaccagaaatcttaggccaaacacctgagcaacaaccaggccaaaatactaatcaatcaggagctgaaaacggctttggttcttctacaaggcctaatgcatcaactaactccaatcttaatcaacttccacagactggtaatgagcattctaatactgcacttgctggtctagcattggctttcttgactgctatgcttggtttgggcaagaagcgtaaacatgattag

SEQ ID NO: 24 - DNA, 4350 bp, synthetic construct
  misc_feature 1..4350: note = GbpA-MBP Chimeric Sequence
  source 1..4350: mol_type = other DNA
ttgtatttaggagggttaataatgctatcaagaaaaaattataaggaaactatacgaaaacagacacctacaaaacagtactatactattaagaaattaactgttggggttacttcggtattaattggtctatcctttatgggagaactagaaggggatagcgttcatgcggacacgatgacagcaagcagtgagtcaacaagtgttacgtcgacgactgctcaggatggtttaaaaaaatctccacaactctatttgcaagttactgatacaaataacccaagtacaccattaagtgcttcatccacagggactagtaagaatgttacctcatcagctgcggtacaagtgaagtccgctagtgatgaagaagatagtgattctacactagctaagggagaaaataaatttgctcggtcagcagtaaaagattcagtcactgatgggaaaacaagtacagcagaaattaatccggcaaaattaagcagtcctgctttaataacgcaactcaaccaatccttagctaagagcagtacgagtgatgcagcaaaagctaatgatgagttagaaattaaagcaacagatccgactaattatccaaactgtggcgatgtgtatgggccattatttgaattggatgctagcggacagcttgttaataaagatgaagttatatctcttaaagatatgtatattttccaaatattgaaattagtaaatacaaaagatagtgactttcaatatgtaatattaacaatgaatcgtaaagatactgcagataggtctgtatatctttttgtaactggaagcaattatagtaatgctgttgttgttaaagtaaagccaaatgatacttatgaattaagtaaaactggatatagtgttacttatacagaaccaacaactataaatggacattatgttgatggaactttttatgttacaggaagtacttacgatgatggttttataatgccagattggcaactgcagcaccttcagattatatatagtttaggaaattatgatccaagcaatactgacgcaacatcagtttgtgaaataatgccaagttatgaaaaggtaccggtaattaaatatagtggagtaccttcaaatattagccaacctaaggtttacattaccgggtttacgggtcaagagtttaacgttacagatattattaacaattataagaaagtttttaagggctactatcttcaaaatcctaatgtggcgtccatgggaactctttcccaatttgagaatggtggttattacttaaagacatattatgataatgatggtaatgttgactttaagggcttgtatcatcaaattgatgatcagggaacaatgagtgtgagtgttcttaatgcagataataaaacaattgttggacctgaaaatattcttgctggtaaatcgcataactttaactttaatggtcataactggattgcgcggaatccttatgtcactagttcagctcacgaagtcatattaaagtatgctaagttaggttcagttattcctgttgatgaaaacggaaataaaataaacgatggatggcaatatgttaatgatccagatgatgcttccaaagccactagcccatatgaaaaagcgccagttatcgatggttatgtagctgtaaatccagatgaaacgatcgttcttcctcataacttaagtagtgacacaaagatttattaccgaaagaggattggtagtgctggtagtgctgaagctggtagtaattggagtcatccacaatttgaaaaaggtagtgctggtagtgctgctggtagtcacggttacgtatcggcagttgaaaacggtgtagccgaagggcgtgtaactctttgtaaatttgcagccaacggtacaggggagaaaaacacacactgtggtgcaattcaatatgaacctcaatctgtagaaggtcctgatggtttccctgtaacaggtcctcgtgatggtaaaattgcctctgcagaatctgcccttgcagccgcacttgatgaacaaactgcagaccgttgggtcaagcgtcctattcaagcaggtcctcaaactttcgagtggaccttcactgcaaaccacgtaacgaaggattggaagtactacattactaagccaaactggaacccaaaccagcctcttagccgtgatgcatttgacttgaaccctttctgtgtcgtagaagggaacatggttcagcctcctaagcgtgtatctcacgaatgtattgttcctgaacgtgaagggtaccaggtaatcctagcagtctgggatgtaggtgatactgcagcctcgttctacaacgttattgacgttaagtttgacggtggtagtgctggtagtgctgctggtagtggtgaatttaaagttacctatagtggtagtgacagcaagacctacgatggtaacccagctaacttcgagccaacgacagttcagtggagtggcttgaaaggactgaacacttcaaccttaacgtccgctgacttcacgtggaatactgcggataagaaggcaccaacggatgccggtaagtacacacttagtttgaatacgaccggagaagcagccttacgtaaggctaacccgaactatgatctcaagacaattagcggtagttacacctacacgattaatccactagggattgataaagttacctatagtggtagtgacagcaagacctacgatggtaacccagctaacttcgagccaacgacagttcagtggagtggcttgaaaggactgaacacttcaaccttaacgtccgctgacttcacgtggaatactgcggataagaaggcaccaacggatgccggtaagtacacacttagtttgaatacgaccggagaagcagccttacgtaaggctaacccgaactatgatctcaagacaattagcggtagttacacctacacgattaatccactagggattgataaagttacctatagtggtagtgacagcaagacctacgatggtaacccagctaacttcgagccaacgacagttcagtggagtggcttgaaaggactgaacacttcaaccttaacgtccgctgacttcacgtggaatactgcggataagaaggcaccaacggatgccggtaagtacacacttagtttgaatacgaccggagaagcagccttacgtaaggctaacccgaactatgatctcaagacaattagcggtagttacacctacacgattaatccactagggattgataaagttacctatagtggtagtgacagcaagacctacgatggtaacccagctaacttcgagccaacgacagttcagtggagtggcttgaaaggactgaacacttcaaccttaacgtccgctgacttcacgtggaatactgcggataagaaggcaccaacggatgccggtaagtacacacttagtttgaatacgaccggagaagcagccttacgtaaggctaacccgaactatgatctcaagacaattagcggtagttacacctacacgattaatccactagggattgataaagttacctatagtggtagtgacagcaagacctacgatggtaacccagctaacttcgagccaacgacagttcagtggagtggcttgaaaggactgaacacttcaaccttaacgtccgctgacttcacgtggaatactgcggataagaaggcaccaacggatgccggtaagtacacacttagtttgaatacgaccggagaagcagccttacgtaaggctaacccgaactatgatctcaagacaattagcggtagttacacctacacgattaatccactagggattgtgactgtaaattacaagggctatgataagaaagtctatgatggtcaacctggaacgattaatccgggtaaattaacgtggagtaagttgccagatggtacttcattgaagatgccaacatggagtatagatgatttcgcttgggaaacagctgatggcttagcaccaacggcagtaggaacttatcggattatcttgacggatgctggtaaggctgcactaaagaagattaatccaaattatgacttaagcagtattactggtgtctttacttatgaaattaagccagcacagacaccagaaatcttaggccaaacacctgagcaacaaccaggccaaaatactaatcaatcaggagctgaaaacggctttggttcttctacaaggcctaatgcatcaactaactccaatcttaatcaacttccacagactggtaatgagcattctaatactgcacttgctggtctagcattggctttcttgactgctatgcttggtttgggcaagaagcgtaaacatgattag

SEQ ID NO: 25 - DNA, 7373 bp, Salmonella enterica
  source 1..7373: mol_type = genomic DNA
ttattcatggctcatacgttgttcgtattctggtctctggcgaggccattttttcgaaacgcctaatcagttccgccaggctaccggcctgcattttttccatgactctggcgcggtgcacctctacggtacgcaccgcgatattcatcgcttccgcaatttcacggttcataaatccttttgccaccaggctggccagctcacgctctttcggcgtcaactgctggtaacacagtataatctcacgacgcgccaccgctgccgatgaaaccgtcagcgcacgctccagcgccgcctgtagcggttttaccgataccggtttttgcagaaaatcgacggcgccgcgtttcatctgctccacggccatcggtacatcgccatgcccggtaagaaaaacaaccgccagggtacttccgcactggcgcaacgcatcatgaacgccctgcccatccagtaccggcattcgcatatccagtaatacgaccccggcctgatacagactggcctgcgccaaaaaatccgccccctgcgtccagcattttacgtcatatcccagactttccagtaaaaacgcgcacgcgttagtgaccgccgtatcatcatccagtagatgaattgtcgccatccctgcccccattttcatgtaagaaatgtatcgtaaccaccgttcccgacagaccgtccggcgcggtctggttcctgatgctgatatcgccccgcccataccgcaccagccgctggcaaatcgccagccctaagcccatcccctctttacgggtggtcataaacggctgaaacgcctgacgtaatagcgcctcatcgattcccccggcgttatcctgtaaaacaatactgatgccgttttcagtgcgttcagcaacgatccataaatgggtggcgcccgcctgagccgcattaagaatgatattcgccagcacctgttccagcagcactgacggcagcgttacgcgcagcgcagcgctaacctcggtatgcagagtcactgtcggaaactgttgcgccatacgcaacaattgccagacatgatcaatcgcctcgcgaatggctatggccttccacgcttcggttagcaccgggttgccctgcgcctggctgacccagtgacgcaggttacgcagagtatccgcaccgcgttgcgcctgctggtcaatctgctccagcgccggcagcaagggatgctgttcatctgcagcgcgcagtcgaatcaggcacccctgggcataatgtcgaatcgcggaaagcggctgattaagctcatgggcaaacccggaggtcatttcacccaacacgctcatttgccgggcggtttccagcgcccgctcatgctgatgaagaactacgctattacgttccagttgctttccacgtcgacgcaccagcagcatgacccaaatataattgagcgtgagcaacaagaacgccagaatcacgccgccgaccattagctggtgctggattaaccaacttttgacatccagccacagtcgacgctgctgagggtgctgacgaacatcacgcagcaaggcttccacctgactggtggacgcaggcgcgccccagtgaaatgacgcggcggcgggcgcgttgaatagcgctcgcgttacgcgatccgccagcgcatcgcttaccgcaggtagcgccgcgaacgaccagtcaggatataacggcgtactggttaagcaaggcaggggcgtcggtcgggaaagcagcgcgataaagtcctttttattaatcaatccttcctgatccatattttctaacaggcacactggcacaattgccgcctgcaccgctttttcgcgcagcatatagactaaggcatcgccaggaaatccggtaaaacggagatgaaaatcgcgctccgggcgtaagcccgcgtcgctgagcgctttatagcctaataaatagccgccaaacgcctgagcatcaatcgcgccgacggtcttaccgatgagatcatgcgccgtggtgatgccgctatcgcgccgggtcaaaatcacgctgccaataacattactcaccgctttcccatcgcgcgtggagcgcagggaagctaaccagcgcagcggcgcatggctgttcagttggacaaattgcgccgggttggttatcacaaactgcacggttccctggttaacggcctcctgcatttgatgcagatccagcggctggatgtgaaaggtttcgcctggaagctgttggcttaatgtctttgccaacggttgccagtggctacgcgtagacgcctcgccgcgcatggccaaaataccgatattccacgtccctgcccacgcgccatgacaaagtagccctactgccgccaacaccgccaggcgccttacggttttacctctcaccccaatatccctgtcaattatgttgttttagatcaacaacaagccgggtatgtggttaaccacaatagagcgcaccccgcctcgatttttacactgtaaatcatcgacattttttattcattacacatgaaccaacatcgtgacaaatgtttcattgttggcaatgtggacgggagtcaatatggacagcagtaaacggcaatttctccagcagcttggcgtcctgaccgctggcgcctcgctggttccgctggctgaagcgaaatttcctttttcgccggagcggcatgaaggctctccccgacaccgttacgccatgcttatcgatctgcggcgttgtatcggctgtcagtcctgtaccgtaagttgcactattgaaaaccaaacgccgcaaggcgcgtttcgtacgacggtgaaccaataccaggtccagcgtgaaggtagtcaggaagtcacgaatgtgctgttgccgcgtctgtgcaaccattgcgataaccccccctgtgtgccggtctgcccggtacaagccacctttcagcgggaagatggcattgtggtggtggataacaaacgctgcgtcggctgcgcctattgtgtccaggcgtgtccttacgacgcccgatttatcaatcatgaaacgcaaactgccgataaatgcacgttttgcgtccatcgtctggaagccggactgttacccgcttgcgtagagtcctgcgtcggcggcgcgcgtattattggcgatatcaaagatccccatagccgcatcgccaccatgcttcatcagcatcgcgacgctatcaaggtattaaagccggaaaacggcacgtcgccccatgttttctacctgggtctggacgacgcctttgtcaccccattaatgggccgtgcgcagcccgcgctttggcaggaggtctgaatgacgcattcactcatcattgaagaagtgctggctcacccgcaggacattagctggctgccgtgggcggtacaatatttcttttttattggcattgccgcctgcgccgcactgtttgcctgttatcttcactggcggaaaaaagacgccgcaacagaagaaaatcgggcattactgattgccattacctgtgcgattaccgcaccgctggcgctgacggcggatctgcaccagaccgcccgcgtctggcatttctatgcctggccgacgccctggtcgtggatgccctggggagcgttattcctgccgctgtttaccggatttctcgctctgtggttcctggcgcagcagattaaacgattattcaataaaagttacaacgtcactaaatggttggcgttagccagcgcgctttgcgcggtgggcctgttgatttataccggccgcgaagtctccgttgtgctggcgcgcccaatctggtttagctacgccttccccgtggcgatgtttcttagcgccttacaggcgttcttcgcgctgatgattgtcgccgcccgacgcgactcggtaaggctgccaaaaatattgtggggacaaatctggacgctggcggcgctggggctggttgtggccatgtgggttagcggcgatacgctttccggcacggcaatccgtcagtggattaccgtcgccctgtcagccaaatattacgctgtcggctgggtagcgctgtgggtatgcacactgctgttctgtagcctggcgctacgccatccgttatcacagctaagacgcgtcctgctggttctcagcgcgctggcgctatgttggctgatgcgctggacattgttgattcaggtacaaaccgtccccaagttcaacgcgcaatttaacccttactcgttaccaggcggaacggatggctggctggctattctcggcaccttcggcctgtggatagcgctactgattattattcgtgaaacgctgaacggactcaccaggagattacaacatggctaatttaacccgtcgtcagtggctaaaagtcggtctcgccgtcggtgggatggtcacttttggtctgagctaccgtgatgtggcgaaacgcgcaattgatggcctgttaaacgggacgtccggcaaggtaacgcgcgaccgcatctttggcaatgcgttaattccggaggcgcaggcgcaaacacactggcagcaaaatccacaacaaaccatcgccatgacgcaatgcttcggctgttggacacagtgcggtatccgcgcccgggttaatgccgatggcaaagtgatacgcatcgccggcaatccctatcaccccttgtcgcaggaacacccgattgactcgtccgtcccttttagcgaagccatggagcaactggcgggagaaagcggtcttgacgcccgctcaaccgcctgcgcgcgcggcgccacgctgctggaaagcctgtacagtccgctacgactgcttgaaccgatgaaacgcgtgggtaaacgcggcgaagggaaatggcagcgcatcagctttgagcaacttattgaagaagtcgtggaaggcggcgatctgtttggcgaaggtcatgtggacggactgcgcgctattcatgcgccggatacgccaattgacgcaaagcaccccagtttcgggcccaaaaccaatcagttactggtcacgaataccagcgacgaaggccgcgatgcgtttctgcgtcgttttgcgctaaatagcttcggcagcaagaatttcggcgcgcatggcgcctactgtggactggcttaccgggccggctccggggcattgatgggcgatctggataaaaacccgcatgtcaaacccgactgggaaaacgtggagtttgcgctctttatgggcacctccccggcacagtccggcaatccgtttaaacgccaggcacgtcagttggcgagcgcccgactgcgtgagaattttcaatacgtcgtggtcgcccccgccctccccttatcaacggtgctcgccgatcctcgcggtcgctggcaaccggtcatgcccggcagtgattcggcgctggcaatggggatgatccgctggatcatggataatcaacgttataatgctgattatctggcgattcccggcgtacaggcgatgcagcaggccggcgagcaaagttggaccaacgccacgcacctggtcattgcggatgagctgccgacgcttgccggacaacacctgacgctgcgccatcttacgcccgatggcgaagagacccctgtcgtactgaataccgacggcgagttggtcgatgcgtccacttgccgacaggcacggcttttcgtgacgcagtacgttacgctcgccgacggccaacgggtcacggtgaagagcgggttgcaacgcctgaaagaggcggcagaaaagctctcgttggcgcaatacagcgaacagtgcggcgtgccggaagcgcaaattatcgcgctggcggaaacctttaccagtcacggacgtaaagctgcggtcatcagtcacggcggcatgatggccggcaatgggttttataacgcctggtcggtcatgatgcttaacgcgctgatcggcaacctcagcttgtccggcggcgtctttgtcggcggcggcaaattcaacggcgttagcgacggcccccgctacaacatgaacagttttgccggaaaagtgaaaccgtccgggttaagtattgcccgtagcaaaaccgcttatgaagcatcggaagaataccgcgacaaaattgccggtgggcaatccccttatccagccaaagcgccgtggtatccctttgtggcaggccagcttaccgaactgttgacctccgcgctcgaaggctatccttatccgcttaaagcctggatttccaatatgagcaacccgttttacggtgttcccggtctacgcgccgtggcggaagaaaaactaaaagaccctcgccgactgccgctctttatcgcgattgacgcctttatgaatgaaacgacggcgctggcggattacattgtgccggatacgcacaattttgagagctggggctttacggcgccctggggcggcgtagccagtaaagccactaccgcccgctggccggttgtcgcccccgccactcaccgcacggcggacgggcaacctgtctcaatggaagcattttgtattgcggtagcaaaacggctccatctgcccggcttcggcgaccgggcgataaccgatccgcagggcaatacttttccactgaaccgggcggaagacttctatctgcgcgtagccgctaatatcgcctttatgggcaagacgccggtcgcgctggcaaatcaggaagatatttcgcttaccggcgtcagccgcattctgccagcaattcagcacacgcttaaagctgatgaggtcggtcgcgtggcgtttatctactcgcgtggcggccggtttgcgcccgaggatagcggctatacggagcaacggttaggtaacgcgtggaaaaaacccttacagatctggaatgcagatgtcgccgcccaccgtcacgccatcaccggggagcgcttcagcggttgcccggtctggtatccggcgcgtttgtcagatggtcgtgcgattgacgaccagtttcccattgggcaatggccgctgaaactgatttcatttaaatcaaataccatgtccagctcaacagccgtcatcccgcgcttacaccatgtgaagccagcaaacctggtggcgctgaatccgcaagacggcgagcgttatggactgcaacatggcgatcgggtacggatcattacgccgggcggtcaggtcgtggcgcaaatcagtttgttaaatggcgtgatgccaggcgtcatcgccatcgaacacggatatggccaccgcgagatgggcgcaacgcagcactctctggatggcgtgcctatgccgtatgatccacaaatcagggcaggcataaatcttaacgatctgggctttgccgatccgacaagaaccattaccaacacctggctcgactgggtttctggcgcggcagtacgtcaggggctgccggcaaaaatcgagcgtatataac

SEQ ID NO: 26 - DNA, 1458 bp, Vibrio cholerae
  source 1..1458: mol_type = genomic DNA
atgaaaaaacaacctaaaatgaccgctattgccctgatcctctctggtatcagtggattagcgtatggacacggctacgtttccgcagtggaaaacggtgtcgccgaaggacgtgtcaccttgtgtaaatttgccgctaacggcactggagagaaaaacactcactgtggcgcgattcaatacgaaccacaaagtgtcgaaggcccagatggcttcccggtcactggccctcgtgatggcaaaattgccagtgcggaatcggcactggcggcagcgctggatgagcaaaccgccgaccgttgggtaaagcgcccaattcaagctggcccacaaaccttcgagtggacgttcaccgccaaccacgtcacaaaggattggaaatactacattaccaaaccaaactggaacccaaaccagccattgtcgcgtgatgcatttgacctcaatccgttctgtgtcgttgaaggaaatatggtgcagccaccaaaacgtgtcagccacgaatgtatcgtgcctgagcgcgaagggtatcaggtcatcctcgccgtatgggatgttggcgataccgcagcttccttctacaacgtgatcgacgtgaaatttgacggtaacggcccagtgttacccgattggaacccagcaggtcaaatcattccaagtatggatctcagcattggcgataccgtgtacactcgcgtgtttgataacgatggggaaaaccctgcttatcgcactgagctaaaaattgactctgagacgctaaccaaagccaatcaatggtcttacgctctggcgactaaaattaaccaaacgcaaaaacagcaacgtgctggtcagcttaatggcgatcaatttgttcccgtttacggcaccaacccgatttatctgaaagaaggcagtggcttgaagagtgttgaaattggctaccaaattgaagcgccacagcctgagtattcactgacggtttctggtctagcgaaagagtatgagattggcgaacaaccgattcagcttgacctgactttagaagcgcaaggtgaaatgagcgcagagctgaccgtgtataaccaccaccaaaaaccgctggcaagttggtcacaagcgatgacggatggcgagctgaaatccatcacgctagagctgagcgaagctaaagcgggacatcatatgttggtttctcgcatcaaagatcgcgatggcaatctgcaagatcaacaaactctcgatttcatgctggttgaaccgcaaacaccaccaacaccgggtgactacgactttgtgttcccgaatggcctgaaagagtacgtggctggcaccaaagtgctcgctagtgatggcgcaatctaccaatgtaagccatggccatactctggctactgccagcaatggacaagtaacgctactcaataccaaccgggtactggcagtcattgggaaatggcgtgggataaacgttaa

SEQ ID NO: 27 - DNA, 540 bp, Vibrio cholerae
  source 1..540: mol_type = genomic DNA
atgaaaaaacaacctaaaatgaccgctattgccctgatcctctctggtatcagtggattagcgtatggacacggctacgtttccgcagtggaaaacggtgtcgccgaaggacgtgtcaccttgtgtaaatttgccgctaacggcactggagagaaaaacactcactgtggcgcgattcaatacgaaccacaaagtgtcgaaggcccagatggcttcccggtcactggccctcgtgatggcaaaattgccagtgcggaatcggcactggcggcagcgctggatgagcaaaccgccgaccgttgggtaaagcgcccaattcaagctggcccacaaaccttcgagtggacgttcaccgccaaccacgtcacaaaggattggaaatactacattaccaaaccaaactggaacccaaaccagccattgtcgcgtgatgcatttgacctcaatccgttctgtgtcgttgaaggaaatatggtgcagccaccaaaacgtgtcagccacgaatgtatcgtgcctgagcgcgaagggtatcaggtcatc

SEQ ID NO: 28 - protein, 1222 aa, Lactobacillus reuteri
MLSRKNYKETIRKQTPTKQYYTIKKLTVGVTSVLIGLSFMGELEGDSVHADTMTASSESTSVTSTTAQDGLKKSPQLYLQVTDTNNPSTPLSASSTGTSKNVTSSAAVQVKSASDEEDSDSTLAKGENKFARSAVKDSVTDGKTSTAEINPAKLSSPALITQLNQSLAKSSTSDAAKANDELEIKATDPTNYPNCGDVYGPLFELDASGQLVNKDEVISLKDMYIFQILKLVNTKDSDFQYVILTMNRKDTADRSVYLFVTGSNYSNAVVVKVKPNDTYELSKTGYSVTYTEPTTINGHYVDGTFYVTGSTYDDGFIMPDWQLQHLQIIYSLGNYDPSNTDATSVCEIMPSYEKVPVIKYSGVPSNISQPKVYITGFTGQEFNVTDIINNYKKVFKGYYLQNPNVASMGTLSQFENGGYYLKTYYDNDGNVDFKGLYHQIDDQGTMSVSVLNADNKTIVGPENILAGKSHNFNFNGHNWIARNPYVTSSAHEVILKYAKLGSVIPVDENGNKINDGWQYVNDPDDASKATSPYEKAPVIDGYVAVNPDETIVLPHNLSSDTKIYYRKRIKVTYSGSDSKTYDGNPANFEPTTVQWSGLKGLNTSTLTSADFTWNTADKKAPTDAGKYTLSLNTTGEAALRKANPNYDLKTISGSYTYTINPLGIDKVTYSGSDSKTYDGNPANFEPTTVQWSGLKGLNTSTLTSADFTWNTADKKAPTDAGKYTLSLNTTGEAALRKANPNYDLKTISGSYTYTINPLGIDKVTYSGSDSKTYDGNPANFEPTTVQWSGLKGLNTSTLTSADFTWNTADKKAPTDAGKYTLSLNTTGEAALRKANPNYDLKTISGSYTYTINPLGIDKVTYSGSDSKTYDGNPANFEPTTVQWSGLKGLNTSTLTSADFTWNTADKKAPTDAGKYTLSLNTTGEAALRKANPNYDLKTISGSYTYTINPLGIDKVTYSGSDSKTYDGNPANFEPTTVQWSGLKGLNTSTLTSADFTWNTADKKAPTDAGKYTLSLNTTGEAALRKANPNYDLKTISGSYTYTINPLGIVTVNYKGYDKKVYDGQPGTINPGKLTWSKLPDGTSLKMPTWSIDDFAWETADGLAPTAVGTYRIILTDAGKAALKKINPNYDLSSITGVFTYEIKPAQTPEILGQTPEQQPGQNTNQSGAENGFGSSTRPNASTNSNLNQLPQTGNEHSNTALAGLALAFLTAMLGLGKKRKHD

SEQ ID NO: 29 - protein, 1442 aa, synthetic construct
  REGION 1..1442: note = GbpA-MBP Chimeric Sequence
MLSRKNYKETIRKQTPTKQYYTIKKLTVGVTSVLIGLSFMGELEGDSVHADTMTASSESTSVTSTTAQDGLKKSPQLYLQVTDTNNPSTPLSASSTGTSKNVTSSAAVQVKSASDEEDSDSTLAKGENKFARSAVKDSVTDGKTSTAEINPAKLSSPALITQLNQSLAKSSTSDAAKANDELEIKATDPTNYPNCGDVYGPLFELDASGQLVNKDEVISLKDMYIFQILKLVNTKDSDFQYVILTMNRKDTADRSVYLFVTGSNYSNAVVVKVKPNDTYELSKTGYSVTYTEPTTINGHYVDGTFYVTGSTYDDGFIMPDWQLQHLQIIYSLGNYDPSNTDATSVCEIMPSYEKVPVIKYSGVPSNISQPKVYITGFTGQEFNVTDIINNYKKVFKGYYLQNPNVASMGTLSQFENGGYYLKTYYDNDGNVDFKGLYHQIDDQGTMSVSVLNADNKTIVGPENILAGKSHNFNFNGHNWIARNPYVTSSAHEVILKYAKLGSVIPVDENGNKINDGWQYVNDPDDASKATSPYEKAPVIDGYVAVNPDETIVLPHNLSSDTKIYYRKRIGSAGSAEAGSNWSHPQFEKGSAGSAAGSHGYVSAVENGVAEGRVTLCKFAANGTGEKNTHCGAIQYEPQSVEGPDGFPVTGPRDGKIASAESALAAALDEQTADRWVKRPIQAGPQTFEWTFTANHVTKDWKYYITKPNWNPNQPLSRDAFDLNPFCVVEGNMVQPPKRVSHECIVPEREGYQVILAVWDVGDTAASFYNVIDVKFDGGSAGSAAGSGEFKVTYSGSDSKTYDGNPANFEPTTVQWSGLKGLNTSTLTSADFTWNTADKKAPTDAGKYTLSLNTTGEAALRKANPNYDLKTISGSYTYTINPLGIDKVTYSGSDSKTYDGNPANFEPTTVQWSGLKGLNTSTLTSADFTWNTADKKAPTDAGKYTLSLNTTGEAALRKANPNYDLKTISGSYTYTINPLGIDKVTYSGSDSKTYDGNPANFEPTTVQWSGLKGLNTSTLTSADFTWNTADKKAPTDAGKYTLSLNTTGEAALRKANPNYDLKTISGSYTYTINPLGIDKVTYSGSDSKTYDGNPANFEPTTVQWSGLKGLNTSTLTSADFTWNTADKKAPTDAGKYTLSLNTTGEAALRKANPNYDLKTISGSYTYTINPLGIDKVTYSGSDSKTYDGNPANFEPTTVQWSGLKGLNTSTLTSADFTWNTADKKAPTDAGKYTLSLNTTGEAALRKANPNYDLKTISGSYTYTINPLGIVTVNYKGYDKKVYDGQPGTINPGKLTWSKLPDGTSLKMPTWSIDDFAWETADGLAPTAVGTYRIILTDAGKAALKKINPNYDLSSITGVFTYEIKPAQTPEILGQTPEQQPGQNTNQSGAENGFGSSTRPNASTNSNLNQLPQTGNEHSNTALAGLALAFLTAMLGLGKKRKHD

SEQ ID NO: 30 - DNA, 4329 bp, synthetic construct
  misc_feature 1..4329: note = GbpA-MBP Chimeric Sequence
  source 1..4329: mol_type = other DNA
atgctatcaagaaaaaattataaggaaactatacgaaaacagacacctacaaaacagtactatactattaagaaattaactgttggggttacttcggtattaattggtctatcctttatgggagaactagaaggggatagcgttcatgcggacacgatgacagcaagcagtgagtcaacaagtgttacgtcgacgactgctcaggatggtttaaaaaaatctccacaactctatttgcaagttactgatacaaataacccaagtacaccattaagtgcttcatccacagggactagtaagaatgttacctcatcagctgcggtacaagtgaagtccgctagtgatgaagaagatagtgattctacactagctaagggagaaaataaatttgctcggtcagcagtaaaagattcagtcactgatgggaaaacaagtacagcagaaattaatccggcaaaattaagcagtcctgctttaataacgcaactcaaccaatccttagctaagagcagtacgagtgatgcagcaaaagctaatgatgagttagaaattaaagcaacagatccgactaattatccaaactgtggcgatgtgtatgggccattatttgaattggatgctagcggacagcttgttaataaagatgaagttatatctcttaaagatatgtatattttccaaatattgaaattagtaaatacaaaagatagtgactttcaatatgtaatattaacaatgaatcgtaaagatactgcagataggtctgtatatctttttgtaactggaagcaattatagtaatgctgttgttgttaaagtaaagccaaatgatacttatgaattaagtaaaactggatatagtgttacttatacagaaccaacaactataaatggacattatgttgatggaactttttatgttacaggaagtacttacgatgatggttttataatgccagattggcaactgcagcaccttcagattatatatagtttaggaaattatgatccaagcaatactgacgcaacatcagtttgtgaaataatgccaagttatgaaaaggtaccggtaattaaatatagtggagtaccttcaaatattagccaacctaaggtttacattaccgggtttacgggtcaagagtttaacgttacagatattattaacaattataagaaagtttttaagggctactatcttcaaaatcctaatgtggcgtccatgggaactctttcccaatttgagaatggtggttattacttaaagacatattatgataatgatggtaatgttgactttaagggcttgtatcatcaaattgatgatcagggaacaatgagtgtgagtgttcttaatgcagataataaaacaattgttggacctgaaaatattcttgctggtaaatcgcataactttaactttaatggtcataactggattgcgcggaatccttatgtcactagttcagctcacgaagtcatattaaagtatgctaagttaggttcagttattcctgttgatgaaaacggaaataaaataaacgatggatggcaatatgttaatgatccagatgatgcttccaaagccactagcccatatgaaaaagcgccagttatcgatggttatgtagctgtaaatccagatgaaacgatcgttcttcctcataacttaagtagtgacacaaagatttattaccgaaagaggattggtagtgctggtagtgctgaagctggtagtaattggagtcatccacaatttgaaaaaggtagtgctggtagtgctgctggtagtcacggttacgtatcggcagttgaaaacggtgtagccgaagggcgtgtaactctttgtaaatttgcagccaacggtacaggggagaaaaacacacactgtggtgcaattcaatatgaacctcaatctgtagaaggtcctgatggtttccctgtaacaggtcctcgtgatggtaaaattgcctctgcagaatctgcccttgcagccgcacttgatgaacaaactgcagaccgttgggtcaagcgtcctattcaagcaggtcctcaaactttcgagtggaccttcactgcaaaccacgtaacgaaggattggaagtactacattactaagccaaactggaacccaaaccagcctcttagccgtgatgcatttgacttgaaccctttctgtgtcgtagaagggaacatggttcagcctcctaagcgtgtatctcacgaatgtattgttcctgaacgtgaagggtaccaggtaatcctagcagtctgggatgtaggtgatactgcagcctcgttctacaacgttattgacgttaagtttgacggtggtagtgctggtagtgctgctggtagtggtgaatttaaagttacctatagtggtagtgacagcaagacctacgatggtaacccagctaacttcgagccaacgacagttcagtggagtggcttgaaaggactgaacacttcaaccttaacgtccgctgacttcacgtggaatactgcggataagaaggcaccaacggatgccggtaagtacacacttagtttgaatacgaccggagaagcagccttacgtaaggctaacccgaactatgatctcaagacaattagcggtagttacacctacacgattaatccactagggattgataaagttacctatagtggtagtgacagcaagacctacgatggtaacccagctaacttcgagccaacgacagttcagtggagtggcttgaaaggactgaacacttcaaccttaacgtccgctgacttcacgtggaatactgcggataagaaggcaccaacggatgccggtaagtacacacttagtttgaatacgaccggagaagcagccttacgtaaggctaacccgaactatgatctcaagacaattagcggtagttacacctacacgattaatccactagggattgataaagttacctatagtggtagtgacagcaagacctacgatggtaacccagctaacttcgagccaacgacagttcagtggagtggcttgaaaggactgaacacttcaaccttaacgtccgctgacttcacgtggaatactgcggataagaaggcaccaacggatgccggtaagtacacacttagtttgaatacgaccggagaagcagccttacgtaaggctaacccgaactatgatctcaagacaattagcggtagttacacctacacgattaatccactagggattgataaagttacctatagtggtagtgacagcaagacctacgatggtaacccagctaacttcgagccaacgacagttcagtggagtggcttgaaaggactgaacacttcaaccttaacgtccgctgacttcacgtggaatactgcggataagaaggcaccaacggatgccggtaagtacacacttagtttgaatacgaccggagaagcagccttacgtaaggctaacccgaactatgatctcaagacaattagcggtagttacacctacacgattaatccactagggattgataaagttacctatagtggtagtgacagcaagacctacgatggtaacccagctaacttcgagccaacgacagttcagtggagtggcttgaaaggactgaacacttcaaccttaacgtccgctgacttcacgtggaatactgcggataagaaggcaccaacggatgccggtaagtacacacttagtttgaatacgaccggagaagcagccttacgtaaggctaacccgaactatgatctcaagacaattagcggtagttacacctacacgattaatccactagggattgtgactgtaaattacaagggctatgataagaaagtctatgatggtcaacctggaacgattaatccgggtaaattaacgtggagtaagttgccagatggtacttcattgaagatgccaacatggagtatagatgatttcgcttgggaaacagctgatggcttagcaccaacggcagtaggaacttatcggattatcttgacggatgctggtaaggctgcactaaagaagattaatccaaattatgacttaagcagtattactggtgtctttacttatgaaattaagccagcacagacaccagaaatcttaggccaaacacctgagcaacaaccaggccaaaatactaatcaatcaggagctgaaaacggctttggttcttctacaaggcctaatgcatcaactaactccaatcttaatcaacttccacagactggtaatgagcattctaatactgcacttgctggtctagcattggctttcttgactgctatgcttggtttgggcaagaagcgtaaacatgattag

SEQ ID NO: 31 - DNA, 4991 bp, Salmonella enterica
  source 1..4991: mol_type = genomic DNA
cccaatatccctgtcaattatgttgttttagatcaacaacaagccgggtatgtggttaaccacaatagagcgcaccccgcctcgatttttacactgtaaatcatcgacattttttattcattacacatgaaccaacatcgtgacaaatgtttcattgttggcaatgtggacgggagtcaatatggacagcagtaaacggcaatttctccagcagcttggcgtcctgaccgctggcgcctcgctggttccgctggctgaagcgaaatttcctttttcgccggagcggcatgaaggctctccccgacaccgttacgccatgcttatcgatctgcggcgttgtatcggctgtcagtcctgtaccgtaagttgcactattgaaaaccaaacgccgcaaggcgcgtttcgtacgacggtgaaccaataccaggtccagcgtgaaggtagtcaggaagtcacgaatgtgctgttgccgcgtctgtgcaaccattgcgataaccccccctgtgtgccggtctgcccggtacaagccacctttcagcgggaagatggcattgtggtggtggataacaaacgctgcgtcggctgcgcctattgtgtccaggcgtgtccttacgacgcccgatttatcaatcatgaaacgcaaactgccgataaatgcacgttttgcgtccatcgtctggaagccggactgttacccgcttgcgtagagtcctgcgtcggcggcgcgcgtattattggcgatatcaaagatccccatagccgcatcgccaccatgcttcatcagcatcgcgacgctatcaaggtattaaagccggaaaacggcacgtcgccccatgttttctacctgggtctggacgacgcctttgtcaccccattaatgggccgtgcgcagcccgcgctttggcaggaggtctgaatgacgcattcactcatcattgaagaagtgctggctcacccgcaggacattagctggctgccgtgggcggtacaatatttcttttttattggcattgccgcctgcgccgcactgtttgcctgttatcttcactggcggaaaaaagacgccgcaacagaagaaaatcgggcattactgattgccattacctgtgcgattaccgcaccgctggcgctgacggcggatctgcaccagaccgcccgcgtctggcatttctatgcctggccgacgccctggtcgtggatgccctggggagcgttattcctgccgctgtttaccggatttctcgctctgtggttcctggcgcagcagattaaacgattattcaataaaagttacaacgtcactaaatggttggcgttagccagcgcgctttgcgcggtgggcctgttgatttataccggccgcgaagtctccgttgtgctggcgcgcccaatctggtttagctacgccttccccgtggcgatgtttcttagcgccttacaggcgttcttcgcgctgatgattgtcgccgcccgacgcgactcggtaaggctgccaaaaatattgtggggacaaatctggacgctggcggcgctggggctggttgtggccatgtgggttagcggcgatacgctttccggcacggcaatccgtcagtggattaccgtcgccctgtcagccaaatattacgctgtcggctgggtagcgctgtgggtatgcacactgctgttctgtagcctggcgctacgccatccgttatcacagctaagacgcgtcctgctggttctcagcgcgctggcgctatgttggctgatgcgctggacattgttgattcaggtacaaaccgtccccaagttcaacgcgcaatttaacccttactcgttaccaggcggaacggatggctggctggctattctcggcaccttcggcctgtggatagcgctactgattattattcgtgaaacgctgaacggactcaccaggagattacaacatggctaatttaacccgtcgtcagtggctaaaagtcggtctcgccgtcggtgggatggtcacttttggtctgagctaccgtgatgtggcgaaacgcgcaattgatggcctgttaaacgggacgtccggcaaggtaacgcgcgaccgcatctttggcaatgcgttaattccggaggcgcaggcgcaaacacactggcagcaaaatccacaacaaaccatcgccatgacgcaatgcttcggctgttggacacagtgcggtatccgcgcccgggttaatgccgatggcaaagtgatacgcatcgccggcaatccctatcaccccttgtcgcaggaacacccgattgactcgtccgtcccttttagcgaagccatggagcaactggcgggagaaagcggtcttgacgcccgctcaaccgcctgcgcgcgcggcgccacgctgctggaaagcctgtacagtccgctacgactgcttgaaccgatgaaacgcgtgggtaaacgcggcgaagggaaatggcagcgcatcagctttgagcaacttattgaagaagtcgtggaaggcggcgatctgtttggcgaaggtcatgtggacggactgcgcgctattcatgcgccggatacgccaattgacgcaaagcaccccagtttcgggcccaaaaccaatcagttactggtcacgaataccagcgacgaaggccgcgatgcgtttctgcgtcgttttgcgctaaatagcttcggcagcaagaatttcggcgcgcatggcgcctactgtggactggcttaccgggccggctccggggcattgatgggcgatctggataaaaacccgcatgtcaaacccgactgggaaaacgtggagtttgcgctctttatgggcacctccccggcacagtccggcaatccgtttaaacgccaggcacgtcagttggcgagcgcccgactgcgtgagaattttcaatacgtcgtggtcgcccccgccctccccttatcaacggtgctcgccgatcctcgcggtcgctggcaaccggtcatgcccggcagtgattcggcgctggcaatggggatgatccgctggatcatggataatcaacgttataatgctgattatctggcgattcccggcgtacaggcgatgcagcaggccggcgagcaaagttggaccaacgccacgcacctggtcattgcggatgagctgccgacgcttgccggacaacacctgacgctgcgccatcttacgcccgatggcgaagagacccctgtcgtactgaataccgacggcgagttggtcgatgcgtccacttgccgacaggcacggcttttcgtgacgcagtacgttacgctcgccgacggccaacgggtcacggtgaagagcgggttgcaacgcctgaaagaggcggcagaaaagctctcgttggcgcaatacagcgaacagtgcggcgtgccggaagcgcaaattatcgcgctggcggaaacctttaccagtcacggacgtaaagctgcggtcatcagtcacggcggcatgatggccggcaatgggttttataacgcctggtcggtcatgatgcttaacgcgctgatcggcaacctcagcttgtccggcggcgtctttgtcggcggcggcaaattcaacggcgttagcgacggcccccgctacaacatgaacagttttgccggaaaagtgaaaccgtccgggttaagtattgcccgtagcaaaaccgcttatgaagcatcggaagaataccgcgacaaaattgccggtgggcaatccccttatccagccaaagcgccgtggtatccctttgtggcaggccagcttaccgaactgttgacctccgcgctcgaaggctatccttatccgcttaaagcctggatttccaatatgagcaacccgttttacggtgttcccggtctacgcgccgtggcggaagaaaaactaaaagaccctcgccgactgccgctctttatcgcgattgacgcctttatgaatgaaacgacggcgctggcggattacattgtgccggatacgcacaattttgagagctggggctttacggcgccctggggcggcgtagccagtaaagccactaccgcccgctggccggttgtcgcccccgccactcaccgcacggcggacgggcaacctgtctcaatggaagcattttgtattgcggtagcaaaacggctccatctgcccggcttcggcgaccgggcgataaccgatccgcagggcaatacttttccactgaaccgggcggaagacttctatctgcgcgtagccgctaatatcgcctttatgggcaagacgccggtcgcgctggcaaatcaggaagatatttcgcttaccggcgtcagccgcattctgccagcaattcagcacacgcttaaagctgatgaggtcggtcgcgtggcgtttatctactcgcgtggcggccggtttgcgcccgaggatagcggctatacggagcaacggttaggtaacgcgtggaaaaaacccttacagatctggaatgcagatgtcgccgcccaccgtcacgccatcaccggggagcgcttcagcggttgcccggtctggtatccggcgcgtttgtcagatggtcgtgcgattgacgaccagtttcccattgggcaatggccgctgaaactgatttcatttaaatcaaataccatgtccagctcaacagccgtcatcccgcgcttacaccatgtgaagccagcaaacctggtggcgctgaatccgcaagacggcgagcgttatggactgcaacatggcgatcgggtacggatcattacgccgggcggtcaggtcgtggcgcaaatcagtttgttaaatggcgtgatgccaggcgtcatcgccatcgaacacggatatggccaccgcgagatgggcgcaacgcagcactctctggatggcgtgcctatgccgtatgatccacaaatcagggcaggcataaatcttaacgatctgggctttgccgatccgacaagaaccattaccaacacctggctcgactgggtttctggcgcggcagtacgtcaggggctgccggcaaaaatcgagcgtata

SEQ ID NO: 32 - DNA, 2374 bp, Salmonella enterica
  source 1..2374: mol_type = genomic DNA
tcatggctcatacgttgttcgtattctggtctctggcgaggccattttttcgaaacgcctaatcagttccgccaggctaccggcctgcattttttccatgactctggcgcggtgcacctctacggtacgcaccgcgatattcatcgcttccgcaatttcacggttcataaatccttttgccaccaggctggccagctcacgctctttcggcgtcaactgctggtaacacagtataatctcacgacgcgccaccgctgccgatgaaaccgtcagcgcacgctccagcgccgcctgtagcggttttaccgataccggtttttgcagaaaatcgacggcgccgcgtttcatctgctccacggccatcggtacatcgccatgcccggtaagaaaaacaaccgccagggtacttccgcactggcgcaacgcatcatgaacgccctgcccatccagtaccggcattcgcatatccagtaatacgaccccggcctgatacagactggcctgcgccaaaaaatccgccccctgcgtccagcattttacgtcatatcccagactttccagtaaaaacgcgcacgcgttagtgaccgccgtatcatcatccagtagatgaattgtcgccatccctgcccccattttcatgtaagaaatgtatcgtaaccaccgttcccgacagaccgtccggcgcggtctggttcctgatgctgatatcgccccgcccataccgcaccagccgctggcaaatcgccagccctaagcccatcccctctttacgggtggtcataaacggctgaaacgcctgacgtaatagcgcctcatcgattcccccggcgttatcctgtaaaacaatactgatgccgttttcagtgcgttcagcaacgatccataaatgggtggcgcccgcctgagccgcattaagaatgatattcgccagcacctgttccagcagcactgacggcagcgttacgcgcagcgcagcgctaacctcggtatgcagagtcactgtcggaaactgttgcgccatacgcaacaattgccagacatgatcaatcgcctcgcgaatggctatggccttccacgcttcggttagcaccgggttgccctgcgcctggctgacccagtgacgcaggttacgcagagtatccgcaccgcgttgcgcctgctggtcaatctgctccagcgccggcagcaagggatgctgttcatctgcagcgcgcagtcgaatcaggcacccctgggcataatgtcgaatcgcggaaagcggctgattaagctcatgggcaaacccggaggtcatttcacccaacacgctcatttgccgggcggtttccagcgcccgctcatgctgatgaagaactacgctattacgttccagttgctttccacgtcgacgcaccagcagcatgacccaaatataattgagcgtgagcaacaagaacgccagaatcacgccgccgaccattagctggtgctggattaaccaacttttgacatccagccacagtcgacgctgctgagggtgctgacgaacatcacgcagcaaggcttccacctgactggtggacgcaggcgcgccccagtgaaatgacgcggcggcgggcgcgttgaatagcgctcgcgttacgcgatccgccagcgcatcgcttaccgcaggtagcgccgcgaacgaccagtcaggatataacggcgtactggttaagcaaggcaggggcgtcggtcgggaaagcagcgcgataaagtcctttttattaatcaatccttcctgatccatattttctaacaggcacactggcacaattgccgcctgcaccgctttttcgcgcagcatatagactaaggcatcgccaggaaatccggtaaaacggagatgaaaatcgcgctccgggcgtaagcccgcgtcgctgagcgctttatagcctaataaatagccgccaaacgcctgagcatcaatcgcgccgacggtcttaccgatgagatcatgcgccgtggtgatgccgctatcgcgccgggtcaaaatcacgctgccaataacattactcaccgctttcccatcgcgcgtggagcgcagggaagctaaccagcgcagcggcgcatggctgttcagttggacaaattgcgccgggttggttatcacaaactgcacggttccctggttaacggcctcctgcatttgatgcagatccagcggctggatgtgaaaggtttcgcctggaagctgttggcttaatgtctttgccaacggttgccagtggctacgcgtagacgcctcgccgcgcatggccaaaataccgatattccacgtccctgcccacgcgccatgacaaagtagccctactgccgccaacaccgccaggcgccttacggttttacctctcac

SEQ ID NO: 33 - DNA, 3060 bp, Salmonella enterica
  source 1..3060: mol_type = genomic DNA
atggctaatttaacccgtcgtcagtggctaaaagtcggtctcgccgtcggtgggatggtcacttttggtctgagctaccgtgatgtggcgaaacgcgcaattgatggcctgttaaacgggacgtccggcaaggtaacgcgcgaccgcatctttggcaatgcgttaattccggaggcgcaggcgcaaacacactggcagcaaaatccacaacaaaccatcgccatgacgcaatgcttcggctgttggacacagtgcggtatccgcgcccgggttaatgccgatggcaaagtgatacgcatcgccggcaatccctatcaccccttgtcgcaggaacacccgattgactcgtccgtcccttttagcgaagccatggagcaactggcgggagaaagcggtcttgacgcccgctcaaccgcctgcgcgcgcggcgccacgctgctggaaagcctgtacagtccgctacgactgcttgaaccgatgaaacgcgtgggtaaacgcggcgaagggaaatggcagcgcatcagctttgagcaacttattgaagaagtcgtggaaggcggcgatctgtttggcgaaggtcatgtggacggactgcgcgctattcatgcgccggatacgccaattgacgcaaagcaccccagtttcgggcccaaaaccaatcagttactggtcacgaataccagcgacgaaggccgcgatgcgtttctgcgtcgttttgcgctaaatagcttcggcagcaagaatttcggcgcgcatggcgcctactgtggactggcttaccgggccggctccggggcattgatgggcgatctggataaaaacccgcatgtcaaacccgactgggaaaacgtggagtttgcgctctttatgggcacctccccggcacagtccggcaatccgtttaaacgccaggcacgtcagttggcgagcgcccgactgcgtgagaattttcaatacgtcgtggtcgcccccgccctccccttatcaacggtgctcgccgatcctcgcggtcgctggcaaccggtcatgcccggcagtgattcggcgctggcaatggggatgatccgctggatcatggataatcaacgttataatgctgattatctggcgattcccggcgtacaggcgatgcagcaggccggcgagcaaagttggaccaacgccacgcacctggtcattgcggatgagctgccgacgcttgccggacaacacctgacgctgcgccatcttacgcccgatggcgaagagacccctgtcgtactgaataccgacggcgagttggtcgatgcgtccacttgccgacaggcacggcttttcgtgacgcagtacgttacgctcgccgacggccaacgggtcacggtgaagagcgggttgcaacgcctgaaagaggcggcagaaaagctctcgttggcgcaatacagcgaacagtgcggcgtgccggaagcgcaaattatcgcgctggcggaaacctttaccagtcacggacgtaaagctgcggtcatcagtcacggcggcatgatggccggcaatgggttttataacgcctggtcggtcatgatgcttaacgcgctgatcggcaacctcagcttgtccggcggcgtctttgtcggcggcggcaaattcaacggcgttagcgacggcccccgctacaacatgaacagttttgccggaaaagtgaaaccgtccgggttaagtattgcccgtagcaaaaccgcttatgaagcatcggaagaataccgcgacaaaattgccggtgggcaatccccttatccagccaaagcgccgtggtatccctttgtggcaggccagcttaccgaactgttgacctccgcgctcgaaggctatccttatccgcttaaagcctggatttccaatatgagcaacccgttttacggtgttcccggtctacgcgccgtggcggaagaaaaactaaaagaccctcgccgactgccgctctttatcgcgattgacgcctttatgaatgaaacgacggcgctggcggattacattgtgccggatacgcacaattttgagagctggggctttacggcgccctggggcggcgtagccagtaaagccactaccgcccgctggccggttgtcgcccccgccactcaccgcacggcggacgggcaacctgtctcaatggaagcattttgtattgcggtagcaaaacggctccatctgcccggcttcggcgaccgggcgataaccgatccgcagggcaatacttttccactgaaccgggcggaagacttctatctgcgcgtagccgctaatatcgcctttatgggcaagacgccggtcgcgctggcaaatcaggaagatatttcgcttaccggcgtcagccgcattctgccagcaattcagcacacgcttaaagctgatgaggtcggtcgcgtggcgtttatctactcgcgtggcggccggtttgcgcccgaggatagcggctatacggagcaacggttaggtaacgcgtggaaaaaacccttacagatctggaatgcagatgtcgccgcccaccgtcacgccatcaccggggagcgcttcagcggttgcccggtctggtatccggcgcgtttgtcagatggtcgtgcgattgacgaccagtttcccattgggcaatggccgctgaaactgatttcatttaaatcaaataccatgtccagctcaacagccgtcatcccgcgcttacaccatgtgaagccagcaaacctggtggcgctgaatccgcaagacggcgagcgttatggactgcaacatggcgatcgggtacggatcattacgccgggcggtcaggtcgtggcgcaaatcagtttgttaaatggcgtgatgccaggcgtcatcgccatcgaacacggatatggccaccgcgagatgggcgcaacgcagcactctctggatggcgtgcctatgccgtatgatccacaaatcagggcaggcataaatcttaacgatctgggctttgccgatccgacaagaaccattaccaacacctggctcgactgggtttctggcgcggcagtacgtcaggggctgccggcaaaaatcgagcgtata

SEQ ID NO: 34 - protein, 1020 aa, Salmonella enterica
MANLTRRQWLKVGLAVGGMVTFGLSYRDVAKRAIDGLLNGTSGKVTRDRIFGNALIPEAQAQTHWQQNPQQTIAMTQCFGCWTQCGIRARVNADGKVIRIAGNPYHPLSQEHPIDSSVPFSEAMEQLAGESGLDARSTACARGATLLESLYSPLRLLEPMKRVGKRGEGKWQRISFEQLIEEVVEGGDLFGEGHVDGLRAIHAPDTPIDAKHPSFGPKTNQLLVTNTSDEGRDAFLRRFALNSFGSKNFGAHGAYCGLAYRAGSGALMGDLDKNPHVKPDWENVEFALFMGTSPAQSGNPFKRQARQLASARLRENFQYVVVAPALPLSTVLADPRGRWQPVMPGSDSALAMGMIRWIMDNQRYNADYLAIPGVQAMQQAGEQSWTNATHLVIADELPTLAGQHLTLRHLTPDGEETPVVLNTDGELVDASTCRQARLFVTQYVTLADGQRVTVKSGLQRLKEAAEKLSLAQYSEQCGVPEAQIIALAETFTSHGRKAAVISHGGMMAGNGFYNAWSVMMLNALIGNLSLSGGVFVGGGKFNGVSDGPRYNMNSFAGKVKPSGLSIARSKTAYEASEEYRDKIAGGQSPYPAKAPWYPFVAGQLTELLTSALEGYPYPLKAWISNMSNPFYGVPGLRAVAEEKLKDPRRLPLFIAIDAFMNETTALADYIVPDTHNFESWGFTAPWGGVASKATTARWPVVAPATHRTADGQPVSMEAFCIAVAKRLHLPGFGDRAITDPQGNTFPLNRAEDFYLRVAANIAFMGKTPVALANQEDISLTGVSRILPAIQHTLKADEVGRVAFIYSRGGRFAPEDSGYTEQRLGNAWKKPLQIWNADVAAHRHAITGERFSGCPVWYPARLSDGRAIDDQFPIGQWPLKLISFKSNTMSSSTAVIPRLHHVKPANLVALNPQDGERYGLQHGDRVRIITPGGQVVAQISLLNGVMPGVIAIEHGYGHREMGATQHSLDGVPMPYDPQIRAGINLNDLGFADPTRTITNTWLDWVSGAAVRQGLPAKIERI

SEQ ID NO: 35 - DNA, 752 bp, Salmonella enterica
  source 1..752: mol_type = genomic DNA
atgtggacgggagtcaatatggacagcagtaaacggcaatttctccagcagcttggcgtcctgaccgctggcgcctcgctggttccgctggctgaagcgaaatttcctttttcgccggagcggcatgaaggctctccccgacaccgttacgccatgcttatcgatctgcggcgttgtatcggctgtcagtcctgtaccgtaagttgcactattgaaaaccaaacgccgcaaggcgcgtttcgtacgacggtgaaccaataccaggtccagcgtgaaggtagtcaggaagtcacgaatgtgctgttgccgcgtctgtgcaaccattgcgataaccccccctgtgtgccggtctgcccggtacaagccacctttcagcgggaagatggcattgtggtggtggataacaaacgctgcgtcggctgcgcctattgtgtccaggcgtgtccttacgacgcccgatttatcaatcatgaaacgcaaactgccgataaatgcacgttttgcgtccatcgtctggaagccggactgttacccgcttgcgtagagtcctgcgtcggcggcgcgcgtattattggcgatatcaaagatccccatagccgcatcgccaccatgcttcatcagcatcgcgacgctatcaaggtattaaagccggaaaacggcacgtcgccccatgttttctacctgggtctggacgacgcctttgtcaccccattaatgggccgtgcgcagcccgcgctttggcaggaggtctg

SEQ ID NO: 36 - protein, 250 aa, Salmonella enterica
MWTGVNMDSSKRQFLQQLGVLTAGASLVPLAEAKFPFSPERHEGSPRHRYAMLIDLRRCIGCQSCTVSCTIENQTPQGAFRTTVNQYQVQREGSQEVTNVLLPRLCNHCDNPPCVPVCPVQATFQREDGIVVVDNKRCVGCAYCVQACPYDARFINHETQTADKCTFCVHRLEAGLLPACVESCVGGARIIGDIKDPHSRIATMLHQHRDAIKVLKPENGTSPHVFYLGLDDAFVTPLMGRAQPALWQEV

SEQ ID NO: 37 - DNA, 1019 bp, Salmonella enterica
  source 1..1019: mol_type = genomic DNA
atgacgcattcactcatcattgaagaagtgctggctcacccgcaggacattagctggctgccgtgggcggtacaatatttcttttttattggcattgccgcctgcgccgcactgtttgcctgttatcttcactggcggaaaaaagacgccgcaacagaagaaaatcgggcattactgattgccattacctgtgcgattaccgcaccgctggcgctgacggcggatctgcaccagaccgcccgcgtctggcatttctatgcctggccgacgccctggtcgtggatgccctggggagcgttattcctgccgctgtttaccggatttctcgctctgtggttcctggcgcagcagattaaacgattattcaataaaagttacaacgtcactaaatggttggcgttagccagcgcgctttgcgcggtgggcctgttgatttataccggccgcgaagtctccgttgtgctggcgcgcccaatctggtttagctacgccttccccgtggcgatgtttcttagcgccttacaggcgttcttcgcgctgatgattgtcgccgcccgacgcgactcggtaaggctgccaaaaatattgtggggacaaatctggacgctggcggcgctggggctggttgtggccatgtgggttagcggcgatacgctttccggcacggcaatccgtcagtggattaccgtcgccctgtcagccaaatattacgctgtcggctgggtagcgctgtgggtatgcacactgctgttctgtagcctggcgctacgccatccgttatcacagctaagacgcgtcctgctggttctcagcgcgctggcgctatgttggctgatgcgctggacattgttgattcaggtacaaaccgtccccaagttcaacgcgcaatttaacccttactcgttaccaggcggaacggatggctggctggctattctcggcaccttcggcctgtggatagcgctactgattattattcgtgaaacgctgaacggactcaccaggagattacaacatgg

SEQ ID NO: 38 - protein, 340 aa, Salmonella enterica
MTHSLIIEEVLAHPQDISWLPWAVQYFFFIGIAACAALFACYLHWRKKDAATEENRALLIAITCAITAPLALTADLHQTARVWHFYAWPTPWSWMPWGALFLPLFTGFLALWFLAQQIKRLFNKSYNVTKWLALASALCAVGLLIYTGREVSVVLARPIWFSYAFPVAMFLSALQAFFALMIVAARHDSVRLPKILWGQIWTLAALGLVVAMWVSGDTLSGTAIRQWITVALSAKYYAVGWVALWVCTLLFCSLALRHPLSQLRRVLLVLSALALCWLMRWTLLIQVQTVPKFNAQFNPYSLPGGTDGWLAILGTFGLWIALLIIIRETLNGLTRRLQHG

SEQ ID NO: 39 - DNA, 639 bp, Salmonella enterica
  source 1..639: mol_type = genomic DNA
atgaaaatgggggcagggatggcgacaattcatctactggatgatgatacggcggtcactaacgcgtgcgcgtttttactggaaagtctgggatatgacgtaaaatgctggacgcagggggcggattttttggcgcaggccagtctgtatcaggccggggtcgtattactggatatgcgaatgccggtactggatgggcagggcgttcatgatgcgttgcgccagtgcggaagtaccctggcggttgtttttcttaccgggcatggcgatgtaccgatggccgtggagcagatgaaacgcggcgccgtcgattttctgcaaaaaccggtatcggtaaaaccgctacaggcggcgctggagcgtgcgctgacggtttcatcggcagcggtggcgcgtcgtgagattatactgtgttaccagcagttgacgccgaaagagcgtgagctggccagcctggtggcaaaaggatttatgaaccgtgaaattgcggaagcgatgaatatcgcggtgcgtaccgtagaggtgcaccgcgccagagtcatggaaaaaatgcaggccggtagcctggcggaactgattaggcgtttcgaaaaaatggcctcgccagagaccagaatacgaacaacgtatgagccatga

SEQ ID NO: 40 - protein, 212 aa, Salmonella enterica
MKMGAGMATIHLLDDDTAVTNACAFLLESLGYDVKCWTQGADFLAQASLYQAGVVLLDMRMPVLDGQGVHDALRQCGSTLAVVFLTGHGDVPMAVEQMKRGAVDFLQKPVSVKPLQAALERALTVSSAAVARREIILCYQQLTPKERELASLVAKGFMNREIAEAMNIAVRTVEVHRARVMEKMQAGSLAELIRRFEKMASPETRIRTTYEP

SEQ ID NO: 41 - DNA, 1779 bp, Salmonella enterica
  source 1..1779: mol_type = genomic DNA
gtgagaggtaaaaccgtaaggcgcctggcggtgttggcggcagtagggctactttgtcatggcgcgtgggcagggacgtggaatatcggtattttggccatgcgcggcgaggcgtctacgcgtagccactggcaaccgttggcaaagacattaagccaacagcttccaggcgaaacctttcacatccagccgctggatctgcatcaaatgcaggaggccgttaaccagggaaccgtgcagtttgtgataaccaacccggcgcaatttgtccaactgaacagccatgcgccgctgcgctggttagcttccctgcgctccacgcgcgatgggaaagcggtgagtaatgttattggcagcgtgattttgacccggcgcgatagcggcatcaccacggcgcatgatctcatcggtaagaccgtcggcgcgattgatgctcaggcgtttggcggctatttattaggctataaagcgctcagcgacgcgggcttacgcccggagcgcgattttcatctccgttttaccggatttcctggcgatgccttagtctatatgctgcgcgaaaaagcggtgcaggcggcaattgtgccagtgtgcctgttagaaaatatggatcaggaaggattgattaataaaaaggactttatcgcgctgctttcccgaccgacgcccctgccttgcttaaccagtacgccgttatatcctgactggtcgttcgcggcgctacctgcggtaagcgatgcgctggcggatcgcgtaacgcgagcgctattcaacgcgcccgccgccgcgtcatttcactggggcgcgcctgcgtccaccagtcaggtggaagccttgctgcgtgatgttcgtcagcaccctcagcagcgtcgactgtggctggatgtcaaaagttggttaatccagcaccagctaatggtcggcggcgtgattctggcgttcttgttgctcacgctcaattatatttgggtcatgctgctggtgcgtcgacgtggaaagcaactggaacgtaatagcgtagttcttcatcagcatgagcgggcgctggaaaccgcccggcaaatgagcgtgttgggtgaaatgacctccgggtttgcccatgagcttaatcagccgctttccgcgattcgacattatgcccaggggtgcctgattcgactgcgcgctgcagatgaacagcatcccttgctgccggcgctggagcagattgaccagcaggcgcaacgcggtgcggatactctgcgtaacctgcgtcactgggtcagccaggcgcagggcaacccggtgctaaccgaagcgtggaaggccatagccattcgcgaggcgattgatcatgtctggcaattgttgcgtatggcgcaacagtttccgacagtgactctgcataccgaggttagcgctgcgctgcgcgtaacgctgccgtcagtgctgctggaacaggtgctggcgaatatcattcttaatgcggctcaggcgggcgccacccatttatggatcgttgctgaacgcactgaaaacggcatcagtattgttttacaggataacgccgggggaatcgatgaggcgctattacgtcaggcgtttcagccgtttatgaccacccgtaaagaggggatgggcttagggctggcgatttgccagcggctggtgcggtatgggcggggcgatatcagcatcaggaaccagaccgcgccggacggtctgtcgggaacggtggttacgatacatttcttacatgaaaatgggggcagggatggcgacaattcatctactggatga

SEQ ID NO: 42 - protein, 592 aa, Salmonella enterica
MRGKTVRRLAVLAAVGLLCHGAWAGTWNIGILAMRGEASTRSHWQPLAKTLSQQLPGETFHIQPLDLHQMQEAVNQGTVQFVITNPAQFVQLNSHAPLRWLASLRSTRDGKAVSNVIGSVILTRRDSGITTAHDLIGKTVGAIDAQAFGGYLLGYKALSDAGLRPERDFHLRFTGFPGDALVYMLREKAVQAAIVPVCLLENMDQEGLINKKDFIALLSRPTPLPCLTSTPLYPDWSFAALPAVSDALADRVTRALFNAPAAASFHWGAPASTSQVEALLRDVRQHPQQRRLWLDVKSWLIQHQLMVGGVILAFLLLTLNYIWVMLLVRRRGKQLERNSVVLHQHERALETARQMSVLGEMTSGFAHELNQPLSAIRHYAQGCLIRLRAADEQHPLLPALEQIDQQAQRGADTLRNLRHWVSQAQGNPVLTEAWKAIAIREAIDHVWQLLRMAQQFPTVTLHTEVSAALRVTLPSVLLEQVLANIILNAAQAGATHLWIVAERTENGISIVLQDNAGGIDEALLRQAFQPFMTTRKEGMGLGLAICQRLVRYGRGDISIRNQTAPDGLSGTVVTIHFLHENGGRDGDNSSTG

SEQ ID NO: 43 - DNA, 5234 bp, synthetic construct
  misc_feature 1..5234: note = vector
  source 1..5234: mol_type = other DNA
aggcacacgaaaaacaagttaagggatgcagtttatcgggcagcgttgggtcctggccacgggtgcgcatgatcgtgctcctgtcgttgaggacccggctaggctggcggggttgccttactggttagcagaatgaatcaccgatacgcgagcgaacgtgaagcgactgctgctgcaaaacgtctgcgacctgagcaacaacatgaatggtcttcggtttccgtgtttcgtaaagtctggaaacgcggaagtcagcgccctgcaccattatgttccggatctgcatcgcaggatgctgctggctaccctgtggaacacctacatctgtattaacgaagcgctggcattgaccctgagtgatttttctctggtcccgccgcatccataccgccagttgtttaccctcacaacgttccagtaaccgggcatgttcatcatcagtaacccgtatcgtgagcatcctctctcgtttcatcggtatcattacccccatgaacagaaatcccccttacacggaggcatcagtgaccaaacaggaaaaaaccgcccttaacatggcccgctttatcagaagccagacattaacgcttctggagaaactcaacgagctggacgcggatgaacaggcagacatctgtgaatcgcttcacgaccacgctgatgagctttaccgcagctgcctcgcgcgtttcggtgatgacggtgaaaacctctgacacatgcagctcccggagacggtcacagcttgtctgtaagcggatgccgggagcagacaagcccgtcagggcgcgtcagcgggtgttggcgggtgtcggggcgcagccatgacccagtcacgtagcgatagcggagtgtatactggcttaactatgcggcatcagagcagattgtactgagagtgcaccatatgcggtgtgaaataccgcacagatgcgtaaggagaaaataccgcatcaggcgctcttccgcttcctcgctcactgactcgctgcgctcggtcgttcggctgcggcgagcggtatcagctcactcaaaggcggtaatacggttatccacagaatcaggggataacgcaggaaagaacatgtgagcaaaaggccagcaaaaggccaggaaccgtaaaaaggccgcgttgctggcgtttttccataggctccgcccccctgacgagcatcacaaaaatcgacgctcaagtcagaggtggcgaaacccgacaggactataaagataccaggcgtttccccctggaagctccctcgtgcgctctcctgttccgaccctgccgcttaccggatacctgtccgcctttctcccttcgggaagcgtggcgctttctcatagctcacgctgtaggtatctcagttcggtgtaggtcgttcgctccaagctgggctgtgtgcacgaaccccccgttcagcccgaccgctgcgccttatccggtaactatcgtcttgagtccaacccggtaagacacgacttatcgccactggcagcagtcccttaacttacttattaaataatttatagctattgaaaagagataagaattgttcaaagctaatattgtttaaatcgtcaattcctgcatgttttaaggaattgttaaattgattttttgtaaatattttcttgtattctttgttaacccatttcataacgaaataattatacttttgtttatctttgtgtgatattcttgatttttttctacttaatctgataagtgagctattcactttaggtttaggatgaaaatattctcttggaaccatacttaatatagaaatatcaacttctgccattaaaagtaatgccaatgagcgttttgtatttaataatcttttagcaaacccgtattccacgattaaataaatctcattagctatactatcaaaaacaattttgcgtattatatccgtacttatgttataaggtatattaccatatattttataggattggtttttaggaaatttaaactgcaatatatccttgtttaaaacttggaaattatcgtgatcaacaagtttattttctgtagttttgcataatttatggtctatttcaatggcagttacgaaattacacctctttactaattcaagggtaaaatggccttttcctgagccgatttcaaagatattatcatgttcatttaatcttatatttgtcattattttatctatattatgttttgaagtaataaagttttgactgtgttttatatttttctcgttcattataaccctctttaatttggttatatgaattttgcttattaacgattcattataaccacttattttttgtttggttgataatgaactgtgctgattacaaaaatactaaaaatgcccatattttttcctccttataaaattagtataattatagcacgagctctgataaatatgaacatgatgagtgatcgttaaatttatactgcaatcggatgcgattattgaataaaagatatgagagatttatctaatttcttttttcttgtaaaaaaagaaagttcttaaaggttttatagttttggtcgtagagcacacggtttaacgacttaattacgaagtaaataagtctagtgtgttagactttatgaaatctatatacgtttatatatatttattatccgattttttattaaaacgtctcaaaatcgtttctgagacgttttagcgtttatttcgtttagttatcggcataatcgttaaaacaggcgttatcgtagcgtaaaagcccttgagcgtagcgtggctttgcagcgaagatgttgtctgttagattatgaaagccgatgactgaatgaaataataagcgcagcgcccttctatttcggttggaggaggctcaagggagtatgagggaatgaaattccctcatgggtttgattttaaaaattgcttgcaattttgccgagcggtagcgctggaaaatttttgaaaaaaatttggaatttggaaaaaaatggggggaaaggaagcgaattttgcttccgtactacgaccccccattaagtgccgagtgccaatttttgtgccaaaaacgctctatcccaactggctcaagggtttaaggggtttttcaatcgccaacgaatcgccaacgttttcgccaacgttttttataaatctatatttaagtagctttattgttgtttttatgattacaaagtgatacactaactttataaaattatttgattggagttttttaaatggtgatttcagaatcgaaaaaaagagttatgatttctctgacaaaagagcaagataaaaaattaacagatatggcgaaacaaaaaggtttttcaaaatctgcggttgcggcgttagctatagaagaatatgcaagaaaggaatcagaacaaaaaaaataagcgaaagctcgcgtttttagaaggatacgagttttcgctacttgtttttgataaggtaattatatcatggctattaaaaatactaaagctagaaattttggatttttattatatcctgactcaattcctaatgattggaaagaaaaattagagagtttgggcgtatctatggctgtcagtcctttacacgatatggacgaaaaaaaagataaagatacatggaataatagtaatattatacaaaatggaaagcactataaaaaaccacactatcacgttatatatattgcacgaaatcctgtaacaatagaaagcgttaggaacaagattaagcgaaaattggggaatagttcagttgctcatgttgagatacttgattatatcaaaggttcatatgaatatttgactcatgaatcaaaggacgctattgctaagaataaacatatatacgacaaaaaagatattttgaacattaatgattttgatattgaccgctatataacacttgatgaaagccaaaaaagagaattgaagaatttacttttagatatagtggatgactataatttggtaaatacaaaagatttaatggcttttattcgccttaggggagcggagtttggaattttaaatacaaagatattgtttcaacaaagaatgatgtactctagcgcctttagattatggtttgagggcaattatcagtgtggatatagagcaagttatgcaaaggttcttgatgctgaaacgggggaaataaaatgacaaacaaagaaaaagagttatttgctgaaaatgaggaattaaaaaaagaaattaaggacttaaaagagcgtattgaaagatacagagaaatggaagttgaattaagtacaacaatagatttattgagaggagggattattgaataaataaaagccccctgacgaaagtcgaagggggtttttattttggtttgatgttgcgattaatagcaatacaattgcaataaacaaaatgatcttccttcaggttatgaccatctgtgccagttcgtaatgtctggtcaactttccgactctgagaaacttctggaatcgctagagaatttctggaatgggattcaggagtggacagaacgacacggatatatagtggatgtgtcaaaacgcataccattttgaacgatgacctctaataattgttaatcatgttggttacgtatttattaacttctcctagtattagtaattatcatggctgtcatggcgcattaacggaataaagggtgtgcttaaatcgggccattttgcgtaataagaaaaaggattaattatgagcgaattgaattaataataaggtaatagatttacattagaaaatgaaaggggattttatgcgtgagaatgttacagtctatccctggcgaaagggggatgtgctgcaaggcgattaagttgggtaacgccagggttttcccagtcacgacgttgtaaaacgacggccagtgagcgcgcgtaatacgactcactatagggcgaattgggtaccgggccccccctcgaggtcgacggtatcgataagcttgatatcgaattcctgcagcccgggggatccactagttctagagcggccgccaccgcggtggagctccagcttttgttccctttagtgagggttaattgcgcgcttggcgtaatcatggtcatagctgtttcctgtgtgaaattgttatccgctcacaattccacacaacatacgagccggaagcataaagtgtaaagcctggggtgcctaatgagtgagctaactcacattaattgcgttgcgctcactgcccgctttccagtcgggaaacctgtcgtgccag

SEQ ID NO: 44 - DNA, 5234 bp, synthetic construct; identical to SEQ ID NO: 43
  misc_feature 1..5234: note = vector
  source 1..5234: mol_type = other DNA

SEQ ID NO: 45 - DNA, 4500 bp, synthetic construct
  misc_feature 1..4500: note = vector
  source 1..4500: mol_type = other DNA
ttccccttctctgaaaatcaacgggcaggtcactgacttgcccgtttttttatcccttctccacaccgttgagctcgaattctcatgtttgacagcttatcactgatcagtgaattaatggcgatgacgcatcctcacgataatatccgggtaggcgcaatcactttcgtctctactccgttacaaagcgaggctgggtatttcccggcctttctgttatccgaaatccactgaaagcacagcggctggctgaggagataaataataaacgaggggctgtatgcacaaagcatcttctgttgagttaagaacgagtatcgagatggcacatagccttgctcaaattggaatcaggtttgtgccaataccagtagaaacagacgaagaagctagaggtgaatcacgacaaagcgtatcaaaaacgtatggagtagggctctaaactctgtataaaaagtttccagctagctgataacgggaaagaaacagagaagggcacaaatattgtgtactttaatgtgccctttaatttattgattggtggttgaattgtccgtaactttttgatttaagtgcaaatttctaataaattagaacactttcttaaattgtcatttggcatattacgaacaattccgcgtaaaaacgttctgttacgctaaacccttatccagcaggctttcaaggatgtaaaccataacactctgcgaactagtgttacattgcgtgtagctttgagtgggcaactttgtgtacacttttgtgtacccaaaaacaaaaatgtgtacccattcaatgatcaccgacacaaagctcaggaaggcgctcggcaagaaaagagatgatatcgagattatttctgattcgcacgagctttctagacgctcaagttagtataaaaaagctgaacgagaaacgtaaaatgatataaatatcaatatattaaattagattttgcataaaaaacagactacataatactgtaaaacacaacatatgcagtcactatgaatcaactacttagatggtattagtgacctgtaacagactgcgggcccaggttatgctgcttttaagacccactttcacatttaagttgtttttctaatccgcatatgatcaattcaaggccgaataagaaggctggctctgcaccttggtgatcaaataattcgatagcttgtcgtaataatggcggcatactatcagtagtaggtgtttccctttcttctttagcgacttgatgctcttgatcttccaatacgcaacctaaagtaaaatgccccacagcgctgagtgcatataatgcattctctagtgaaaaaccttgttggcataaaaaggctaattgattttcgagagtttcatactgtttttctgtaggccgtgtacctaaatgtacttttgctccatcgcgatgacttagtaaagcacatctaaaacttttagcgttattacgtaaaaaatcttgccagctttccccttctaaagggcaaaagtgagtatggtgcctatctaacatctcaatggctaaggcgtcgagcaaagcccgcttattttttacatgccaatacaatgtaggctgctctacacctagcttctgggcgagtttacgggttgttaaaccttcgattccgacctcattaagcagctctaatgcgctgttaatcactttacttttatctaatctagacatcattaattcctaatttttgttgacactctatcattgatagagttattttaccactccctatcagtgatagagaaaagtgaaatgaatagttcgacaaagatcgcattggtaattacgttactcgatgccatggggattggccttatcatgccagtcttgccaacgttattacgtgaatttattgcttcggaagatatcgctaaccactttggcgtattgcttgcactttatgcgttaatgcaggttatctttgctccttggcttggaaaaatgtctgaccgatttggtcggcgcccagtgctgttgttgtcattaataggcgcatcgctggattacttattgctggctttttcaagtgcgctttggatgctgtatttaggccgtttgctttcagggatcacaggagctactggggctgtcgcggcatcggtcattgccgataccacctcagcttctcaacgcgtgaagtggttcggttggttaggggcaagttttgggcttggtttaatagcggggcctattattggtggttttgcaggagagatttcaccgcatagtcccttttttatcgctgcgttgctaaatattgtcactttccttgtggttatgttttggttccgtgaaaccaaaaatacacgtgataatacagataccgaagtaggggttgagacgcaatcgaattcggtatacatcactttatttaaaacgatgcccattttgttgattatttatttttcagcgcaattgataggccaaattcccgcaacggtgtgggtgctatttaccgaaaatcgttttggatggaatagcatgatggttggcttttcattagcgggtcttggtcttttacactcagtattccaagcctttgtggcaggaagaatagccactaaatggggcgaaaaaacggcagtactgctcgaatttattgcagatagtagtgcatttgcctttttagcgtttatatctgaaggttggttagatttccctgttttaattttattggctggtggtgggatcgctttacctgcattacagggagtgatgtctatccaaacaaagagtcatgagcaaggtgctttacagggattattggtgagccttaccaatgcaaccggtgttattggcccattactgtttactgttatttataatcattcactaccaatttgggatggctggatttggattattggtttagcgttttactgtattattatcctgctatcgatgaccttcatgttaacccctcaagctcaggggagtaaacaggagacaagtgcttagttatttcgtcaccaaatgatgttattccgcgaaatataatgaccctcttgataacccaagagggcattttttacgagacgtcctaattcccatgtcagccgttaagtgttcctgtgtcactgaaaattgctttgagaggctctaagggcttctcagtgcgttacatccctggcttgttgtccacaaccgttaaaccttaaaagctttaaaagccttatatattcttttttttcttataaaacttaaaaccttagaggctatttaagttgctgatttatattaattttattgttcaaacatgagagcttagtacgtgaaacatgagagcttagtacgttagccatgagagcttagtacgttagccatgagggtttagttcgttaaacatgagagcttagtacgttaaacatgagagcttagtacgtgaaacatgagagcttagtacgtactatcaacaggttgaactgctgatcttcagatcctctacgccggacgcatcgtggccggatcttgcggccgcaaaaattaaaaatgaagttttggaggcctcatttggtgacgaaataactaagcacttgtctcctgtttactcccctgagcttgaggggtcaacatgaaggtcattgatagcaggataataatacagtaaaacgctaaaccaataatccaaatccagccatcccaaattggtagtgaatgattataaataacagtaaacagtaatgggccaataacaccggttgcattggtaaggctcaccaataatccctgtaaagcaccttgctcatgactctttgtttggatagacatcactccctgtaatgcaggtaaagcgatcccaccaccagccaataaaattaaaacagggaaatctaaccaaccttcagatataaacgctaaaaaggcaaatgcactactatctgcaataaattcgagcagtactgccgttttttcgccccatttagtggctattcttcctgccacaaaggcttggaatactgagtgtaaaagaccaagacccgctaatgaaaagccaaccatcatgctattccatccaaaacgattttcggtaaatagcacccacaccgttgcgggaatttggcctatcaattcgaaatcaaataatgattttattttgactgatagtgacctgttcgttgcaacaaattgataagcaatgcttttttataatgccaacttagtataaaaaagcaggcttcagagcgatggcccccgatggtagtgtggggtctccccatgcgagagtagggaactgccaggcatcaaataaaacgaaaggctcagtcgaaagactgggcctttcgttttatctgttgtttgtcggtgaacgctctcctgagtaggacaaatccgccgggagcggatttgaacgttgcgaagcaacggcccggagggtggcgggcaggacgcccgccataaactgccaggcatcaaattaagcagaaggccatcctgacggatggcctttttgcgtggccagtgccaagcttgcatgc

SEQ ID NO: 46 - DNA, 10255 bp, synthetic construct
  misc_feature 1..10255: note = vector
  source 1..10255: mol_type = other DNA
ctgcaggtcgactctagaggatccgttatatacgctcgatttttgccggcagcccctgacgtactgccgcgccagaaacccagtcgagccaggtgttggtaatggttcttgtcggatcggcaaagcccagatcgttaagatttatgcctgccctgatttgtggatcatacggcataggcacgccatccagagagtgctgcgttgcgcccatctcgcggtggccatatccgtgttcgatggcgatgacgcctggcatcacgccatttaacaaactgatttgcgccacgacctgaccgcccggcgtaatgatccgtacccgatcgccatgttgcagtccataacgctcgccgtcttgcggattcagcgccaccaggtttgctggcttcacatggtgtaagcgcgggatgacggctgttgagctggacatggtatttgatttaaatgaaatcagtttcagcggccattgcccaatgggaaactggtcgtcaatcgcacgaccatctgacaaacgcgccggataccagaccgggcaaccgctgaagcgctccccggtgatggcgtgacggtgggcggcgacatctgcattccagatctgtaagggttttttccacgcgttacctaaccgttgctccgtatagccgctatcctcgggcgcaaaccggccgccacgcgagtagataaacgccacgcgaccgacctcatcagctttaagcgtgtgctgaattgctggcagaatgcggctgacgccggtaagcgaaatatcttcctgatttgccagcgcgaccggcgtcttgcccataaaggcgatattagcggctacgcgcagatagaagtcttccgcccggttcagtggaaaagtattgccctgcggatcggttatcgcccggtcgccgaagccgggcagatggagccgttttgctaccgcaatacaaaatgcttccattgagacaggttgcccgtccgccgtgcggtgagtggcgggggcgacaaccggccagcgggcggtagtggctttactggctacgccgccccagggcgccgtaaagccccagctctcaaaattgtgcgtatccggcacaatgtaatccgccagcgccgtcgtttcattcataaaggcgtcaatcgcgataaagagcggcagtcggcgagggtcttttagtttttcttccgccacggcgcgtagaccgggaacaccgtaaaacgggttgctcatattggaaatccaggctttaagcggataaggatagccttcgagcgcggaggtcaacagttcggtaagctggcctgccacaaagggataccacggcgctttggctggataaggggattgcccaccggcaattttgtcgcggtattcttccgatgcttcataagcggttttgctacgggcaatacttaacccggacggtttcacttttccggcaaaactgttcatgttgtagcgggggccgtcgctaacgccgttgaatttgccgccgccgacaaagacgccgccggacaagctgaggttgccgatcagcgcgttaagcatcatgaccgaccaggcgttataaaacccattgccggccatcatgccgccgtgactgatgaccgcagctttacgtccgtgactggtaaaggtttccgccagcgcgataatttgcgcttccggcacgccgcactgttcgctgtattgcgccaacgagagcttttctgccgcctctttcaggcgttgcaacccgctcttcaccgtgacccgttggccgtcggcgagcgtaacgtactgcgtcacgaaaagccgtgcctgtcggcaagtggacgcatcgaccaactcgccgtcggtattcagtacgacaggggtctcttcgccatcgggcgtaagatggcgcagcgtcaggtgttgtccggcaagcgtcggcagctcatccgcaatgaccaggtgcgtggcgttggtccaactttgctcgccggcctgctgcatcgcctgtacgccgggaatcgccagataatcagcattataacgttgattatccatgatccagcggatcatccccattgccagcgccgaatcactgccgggcatgaccggttgccagcgaccgcgaggatcggcgagcaccgttgataaggggagggcgggggcgaccacgacgtattgaaaattctcacgcagtcgggcgctcgccaactgacgtgcctggcgtttaaacggattgccggactgtgccggggaggtgcccataaagagcgcaaactccacgttttcccagtcgggtttgacatgcgggtttttatccagatcgcccatcaatgccccggagccggcccggtaagccagtccacagtaggcgccatgcgcgccgaaattcttgctgccgaagctatttagcgcaaaacgacgcagaaacgcatcgcggccttcgtcgctggtattcgtgaccagtaactgattggttttgggcccgaaactggggtgctttgcgtcaattggcgtatccggcgcatgaatagcgcgcagtccgtccacatgaccttcgccaaacagatcgccgccttccacgacttcttcaataagttgctcaaagctgatgcgctgccatttcccttcgccgcgtttacccacgcgtttcatcggttcaagcagtcgtagcggactgtacaggctttccagcagcgtggcgccgcgcgcgcaggcggttgagcgggcgtcaagaccgctttctcccgccagttgctccatggcttcgctaaaagggacggacgagtcaatcgggtgttcctgcgacaaggggtgatagggattgccggcgatgcgtatcactttgccatcggcattaacccgggcgcggataccgcactgtgtccaacagccgaagcattgcgtcatggcgatggtttgttgtggattttgctgccagtgtgtttgcgcctgcgcctccggaattaacgcattgccaaagatgcggtcgcgcgttaccttgccggacgtcccgtttaacaggccatcaattgcgcgtttcgccacatcacggtagctcagaccaaaagtgaccatcccaccgacggcgagaccgacttttagccactgacgacgggttaaattagccatgttgtaatctcctggtgagtccgttcagcgtttcacgaataataatcagtagcgctatccacaggccgaaggtgccgagaatagccagccagccatccgttccgcctggtaacgagtaagggttaaattgcgcgttgaacttggggacggtttgtacctgaatcaacaatgtccagcgcatcagccaacatagcgccagcgcgctgagaaccagcaggacgcgtcttagctgtgataacggatggcgtagcgccaggctacagaacagcagtgtgcatacccacagcgctacccagccgacagcgtaatatttggctgacagggcgacggtaatccactgacggattgccgtgccggaaagcgtatcgccgctaacccacatggccacaaccagccccagcgccgccagcgtccagatttgtccccacaatatttttggcagccttaccgagtcgcgtcgggcggcgacaatcatcagcgcgaagaacgcctgtaaggcgctaagaaacatcgccacggggaaggcgtagctaaaccagattgggcgcgccagcacaacggagacttcgcggccggtataaatcaacaggcccaccgcgcaaagcgcgctggctaacgccaaccatttagtgacgttgtaacttttattgaataatcgtttaatctgctgcgccaggaaccacagagcgagaaatccggtaaacagcggcaggaataacgctccccagggcatccacgaccagggcgtcggccaggcatagaaatgccagacgcgggcggtctggtgcagatccgccgtcagcgccagcggtgcggtaatcgcacaggtaatggcaatcagtaatgcccgattttcttctgttgcggcgtcttttttccgccagtgaagataacaggcaaacagtgcggcgcaggcggcaatgccaataaaaaagaaatattgtaccgcccacggcagccagctaatgtcctgcgggtgagccagcacttcttcaatgatgagtgaatgcgtcattcagacctcctgccaaagcgcgggctgcgcacggcccattaatggggtgacaaaggcgtcgtccagacccaggtagaaaacatggggcgacgtgccgttttccggctttaataccttgatagcgtcgcgatgctgatgaagcatggtggcgatgcggctatggggatctttgatatcgccaataatacgcgcgccgccgacgcaggactctacgcaagcgggtaacagtccggcttccagacgatggacgcaaaacgtgcatttatcggcagtttgcgtttcatgattgataaatcgggcgtcgtaaggacacgcctggacacaataggcgcagccgacgcagcgtttgttatccaccaccacaatgccatcttcccgctgaaaggtggcttgtaccgggcagaccggcacacagggggggttatcgcaatggttgcacagacgcggcaacagcacattcgtgacttcctgactaccttcacgctggacctggtattggttcaccgtcgtacgaaacgcgccttgcggcgtttggttttcaatagtgcaacttacggtacaggactgacagccgatacaacgccgcagatcgataagcatggcgtaacggtgtcggggagagccttcatgccgctccggcgaaaaaggaaatttcgcttcagccagcggaaccagcgaggcgccagcggtcaggacgccaagctgctggagaaattgccgtttactgctgtccatattgactcccgtccacattgccaacaatgaaacatttgtcacgatgttggttcatgtgtaatgaataaaaaatgtcgatgatttacagtgtaaaaatcgaggcggggtgcgctctattgtggttaaccacatacccggcttgttgttgatctaaaacaacataattgacagggatattggggtgagaggtaaaaccgtaaggcgcctggcggtgttggcggcagtagggctactttgtcatggcgcgtgggcagggacgtggaatatcggtattttggccatgcgcggcgaggcgtctacgcgtagccactggcaaccgttggcaaagacattaagccaacagcttccaggcgaaacctttcacatccagccgctggatctgcatcaaatgcaggaggccgttaaccagggaaccgtgcagtttgtgataaccaacccggcgcaatttgtccaactgaacagccatgcgccgctgcgctggttagcttccctgcgctccacgcgcgatgggaaagcggtgagtaatgttattggcagcgtgattttgacccggcgcgatagcggcatcaccacggcgcatgatctcatcggtaagaccgtcggcgcgattgatgctcaggcgtttggcggctatttattaggctataaagcgctcagcgacgcgggcttacgcccggagcgcgattttcatctccgttttaccggatttcctggcgatgccttagtctatatgctgcgcgaaaaagcggtgcaggcggcaattgtgccagtgtgcctgttagaaaatatggatcaggaaggattgattaataaaaaggactttatcgcgctgctttcccgaccgacgcccctgccttgcttaaccagtacgccgttatatcctgactggtcgttcgcggcgctacctgcggtaagcgatgcgctggcggatcgcgtaacgcgagcgctattcaacgcgcccgccgccgcgtcatttcactggggcgcgcctgcgtccaccagtcaggtggaagccttgctgcgtgatgttcgtcagcaccctcagcagcgtcgactgtggctggatgtcaaaagttggttaatccagcaccagctaatggtcggcggcgtgattctggcgttcttgttgctcacgctcaattatatttgggtcatgctgctggtgcgtcgacgtggaaagcaactggaacgtaatagcgtagttcttcatcagcatgagcgggcgctggaaaccgcccggcaaatgagcgtgttgggtgaaatgacctccgggtttgcccatgagcttaatcagccgctttccgcgattcgacattatgcccaggggtgcctgattcgactgcgcgctgcagatgaacagcatcccttgctgccggcgctggagcagattgaccagcaggcgcaacgcggtgcggatactctgcgtaacctgcgtcactgggtcagccaggcgcagggcaacccggtgctaaccgaagcgtggaaggccatagccattcgcgaggcgattgatcatgtctggcaattgttgcgtatggcgcaacagtttccgacagtgactctgcataccgaggttagcgctgcgctgcgcgtaacgctgccgtcagtgctgctggaacaggtgctggcgaatatcattcttaatgcggctcaggcgggcgccacccatttatggatcgttgctgaacgcactgaaaacggcatcagtattgttttacaggataacgccgggggaatcgatgaggcgctattacgtcaggcgtttcagccgtttatgaccacccgtaaagaggggatgggcttagggctggcgatttgccagcggctggtgcggtatgggcggggcgatatcagcatcaggaaccagaccgcgccggacggtctgtcgggaacggtggttacgatacatttcttacatgaaaatgggggcagggatggcgacaattcatctactggatgatgatacggcggtcactaacgcgtgcgcgtttttactggaaagtctgggatatgacgtaaaatgctggacgcagggggcggattttttggcgcaggccagtctgtatcaggccggggtcgtattactggatatgcgaatgccggtactggatgggcagggcgttcatgatgcgttgcgccagtgcggaagtaccctggcggttgtttttcttaccgggcatggcgatgtaccgatggccgtggagcagatgaaacgcggcgccgtcgattttctgcaaaaaccggtatcggtaaaaccgctacaggcggcgctggagcgtgcgctgacggtttcatcggcagcggtggcgcgtcgtgagattatactgtgttaccagcagttgacgccgaaagagcgtgagctggccagcctggtggcaaaaggatttatgaaccgtgaaattgcggaagcgatgaatatcgcggtgcgtaccgtagaggtgcaccgcgccagagtcatggaaaaaatgcaggccggtagcctggcggaactgattaggcgtttcgaaaaaatggcctcgccagagaccagaatacgaacaacgtatgagccatgaataagagctcgaattctcatgtttgacagcttatcactgatcagtgaattaatggcgatgacgcatcctcacgataatatccgggtaggcgcaatcactttcgtctctactccgttacaaagcgaggctgggtatttcccggcctttctgttatccgaaatccactgaaagcacagcggctggctgaggagataaataataaacgaggggctgtatgcacaaagcatcttctgttgagttaagaacgagtatcgagatggcacatagccttgctcaaattggaatcaggtttgtgccaataccagtagaaacagacgaagaagctagaggtgaatcacgacaaagcgtatcaaaaacgtatggagtagggctctaaactctgtataaaaagtttccagctagctgataacgggaaagaaacagagaagggcacaaatattgtgtactttaatgtgccctttaatttattgattggtggttgaattgtccgtaactttttgatttaagtgcaaatttctaataaattagaacactttcttaaattgtcatttggcatattacgaacaattccgcgtaaaaacgttctgttacgctaaacccttatccagcaggctttcaaggatgtaaaccataacactctgcgaactagtgttacattgcgtgtagctttgagtgggcaactttgtgtacacttttgtgtacccaaaaacaaaaatgtgtacccattcaatgatcaccgacacaaagctcaggaaggcgctcggcaagaaaagagatgatatcgagattatttctgattcgcacgggcccatggctaattcccatgtcagccgttaagtgttcctgtgtcactgaaaattgctttgagaggctctaagggcttctcagtgcgttacatccctggcttgttgtccacaaccgttaaaccttaaaagctttaaaagccttatatattcttttttttcttataaaacttaaaaccttagaggctatttaagttgctgatttatattaattttattgttcaaacatgagagcttagtacgtgaaacatgagagcttagtacgttagccatgagagcttagtacgttagccatgagggtttagttcgttaaacatgagagcttagtacgttaaacatgagagcttagtacgtgaaacatgagagcttagtacgtactatcaacaggttgaactgctgatcttcagatcctctacgccggacgcatcgtggccggatcttgcggccgcaaaaattaaaaatgaagttttggaggcctcatttggtgacgaaataactaagcacttgtctcctgtttactcccctgagcttgaggggtcaacatgaaggtcattgatagcaggataataatacagtaaaacgctaaaccaataatccaaatccagccatcccaaattggtagtgaatgattataaataacagtaaacagtaatgggccaataacaccggttgcattggtaaggctcaccaataatccctgtaaagcaccttgctcatgactctttgtttggatagacatcactccctgtaatgcaggtaaagcgatcccaccaccagccaataaaattaaaacagggaaatctaaccaaccttcagatataaacgctaaaaaggcaaatgcactactatctgcaataaattcgagcagtactgccgttttttcgccccatttagtggctattcttcctgccacaaaggcttggaatactgagtgtaaaagaccaagacccgctaatgaaaagccaaccatcatgctattccatccaaaacgattttcggtaaatagcacccacaccgttgcgggaatttggcctatcaattgcgctgaaaaataaataatcaacaaaatgggcatcgttttaaataaagtgatgtacaccgaatttgattgcgtctcaacccctacttcggtatctgtattatcacgtgtatttttggtttcacggaaccaaaacataaccacaaggaaagtgacaatatttagcaacgcagcgataaaaaagggactatgcggtgaaatctctcctgcaaaaccaccaataataggccccgctattaaaccaagcccaaaacttgcccctaaccaaccgaaccacttcacgcgttgagaagctgaggtggtatcggcaatgaccgatgccgcgacagccccagtagctcctgtgatccctgaaagcaaacggcctaaatacagcatccaaagcgcacttgaaaaagccagcaataagtaatccagcgatgcgcctattaatgacaacaacagcactgggcgccgaccaaatcggtcagacatttttccaagccaaggagcaaagataacctgcattaacgcataaagtgcaagcaatacgccaaagtggttagcgatatcttccgaagcaataaattcacgtaataacgttggcaagactggcatgataaggccaatccccatggcatcgagtaacgtaattaccaatgcgatctttgtcgaactattcatttcacttttctctatcactgatagggagtgggaaaataactctatcaatgatagggtgtcaaatcgatggcccccgatggtagtgtggggtctccccatgcgagagtagggaactgccaggcatcaaataaaacgaaaggctcagtcgaaagactgggcctttcgttttatctgttgtttgtcggtgaacgctctcctgagtaggacaaatccgccgggagcggatttgaacgttgcgaagcaacggcccggagggtggcgggcaggacgcccgccataaactgccaggcatcaaattaagcagaaggccatcctgacggatggcctttttgcgtggccagtgccaagcttgcatgc

SEQ ID NO: 47 - DNA, 10465 bp, synthetic construct
  misc_feature 1..10465: note = vector
  source 1..10465: mol_type = other DNA
gacctataaggaaaggccaaacaagaacacggttgcaaaaaccgtgcccttaaatattgaatttctattcagaacactttcttaaattgtcatttggcatattacgaacaattccgcgtaaaaacgttctgttacgctaaacccttatccagcaggctttcaaggatgtaaaccataacactctgcgaactagtgttacattgcgtgtagctttgagtgggcaactttgtgtacacttttgtgtacccaaaaacaaaaatgtgtacccattcaatgatcaccgacacaaagctcaggaaggcgctcggcaagaaaagagatgatatcgagattatttctgattcgcacgggcccatggctaattcccatgtcagccgttaagtgttcctgtgtcactgaaaattgctttgagaggctctaagggcttctcagtgcgttacatccctggcttgttgtccacaaccgttaaaccttaaaagctttaaaagccttatatattcttttttttcttataaaacttaaaaccttagaggctatttaagttgctgatttatattaattttattgttcaaacatgagagcttagtacgtgaaacatgagagcttagtacgttagccatgagagcttagtacgttagccatgagggtttagttcgttaaacatgagagcttagtacgttaaacatgagagcttagtacgtgaaacatgagagcttagtacgtactatcaacaggttgaactgctgatcttcagatcctctacgccggacgcatcgtggccggatcttgcggccgcaaaaattaaaaatgaagttttggaggcctcatttggtgacgaaataactaagcacttgtctcctgtttactcccctgagcttgaggggtcaacatgaaggtcattgatagcaggataataatacagtaaaacgctaaaccaataatccaaatccagccatcccaaattggtagtgaatgattataaataacagtaaacagtaatgggccaataacaccggttgcattggtaaggctcaccaataatccctgtaaagcaccttgctcatgactctttgtttggatagacatcactccctgtaatgcaggtaaagcgatcccaccaccagccaataaaattaaaacagggaaatctaaccaaccttcagatataaacgctaaaaaggcaaatgcactactatctgcaataaattcgagcagtactgccgttttttcgccccatttagtggctattcttcctgccacaaaggcttggaatactgagtgtaaaagaccaagacccgctaatgaaaagccaaccatcatgctattccatccaaaacgattttcggtaaatagcacccacaccgttgcgggaatttggcctatcaattgcgctgaaaaataaataatcaacaaaatgggcatcgttttaaataaagtgatgtacaccgaatttgattgcgtctcaacccctacttcggtatctgtattatcacgtgtatttttggtttcacggaaccaaaacataaccacaaggaaagtgacaatatttagcaacgcagcgataaaaaagggactatgcggtgaaatctctcctgcaaaaccaccaataataggccccgctattaaaccaagcccaaaacttgcccctaaccaaccgaaccacttcacgcgttgagaagctgaggtggtatcggcaatgaccgatgccgcgacagccccagtagctcctgtgatccctgaaagcaaacggcctaaatacagcatccaaagcgcacttgaaaaagccagcaataagtaatccagcgatgcgcctattaatgacaacaacagcactgggcgccgaccaaatcggtcagacatttttccaagccaaggagcaaagataacctgcattaacgcataaagtgcaagcaatacgccaaagtggttagcgatatcttccgaagcaataaattcacgtaataacgttggcaagactggcatgataaggccaatccccatggcatcgagtaacgtaattaccaatgcgatctttgtcgaactattcatttcacttttctctatcactgatagggagtgggaaaataactctatcaatgatagggtgtcaaatcgatggcccccgatggtagtgtggggtctccccatgcgagagtagggaactgccaggcatcaaataaaacgaaaggctcagtcgaaagactgggcctttcgttttatctgttgtttgtcggtgaacgctctcctgagtaggacaaatccgccgggagcggatttgaacgttgcgaagcaacggcccggagggtggcgggcaggacgcccgccataaactgccaggcatcaaattaagcagaaggccatcctgacggatggcctttttgcgtggccagtgccaagcttgcatgcctgcaggtcgactctagaggatccgttatatacgctcgatttttgccggcagcccctgacgtactgccgcgccagaaacccagtcgagccaggtgttggtaatggttcttgtcggatcggcaaagcccagatcgttaagatttatgcctgccctgatttgtggatcatacggcataggcacgccatccagagagtgctgcgttgcgcccatctcgcggtggccatatccgtgttcgatggcgatgacgcctggcatcacgccatttaacaaactgatttgcgccacgacctgaccgcccggcgtaatgatccgtacccgatcgccatgttgcagtccataacgctcgccgtcttgcggattcagcgccaccaggtttgctggcttcacatggtgtaagcgcgggatgacggctgttgagctggacatggtatttgatttaaatgaaatcagtttcagcggccattgcccaatgggaaactggtcgtcaatcgcacgaccatctgacaaacgcgccggataccagaccgggcaaccgctgaagcgctccccggtgatggcgtgacggtgggcggcgacatctgcattccagatctgtaagggttttttccacgcgttacctaaccgttgctccgtatagccgctatcctcgggcgcaaaccggccgccacgcgagtagataaacgccacgcgaccgacctcatcagctttaagcgtgtgctgaattgctggcagaatgcggctgacgccggtaagcgaaatatcttcctgatttgccagcgcgaccggcgtcttgcccataaaggcgatattagcggctacgcgcagatagaagtcttccgcccggttcagtggaaaagtattgccctgcggatcggttatcgcccggtcgccgaagccgggcagatggagccgttttgctaccgcaatacaaaatgcttccattgagacaggttgcccgtccgccgtgcggtgagtggcgggggcgacaaccggccagcgggcggtagtggctttactggctacgccgccccagggcgccgtaaagccccagctctcaaaattgtgcgtatccggcacaatgtaatccgccagcgccgtcgtttcattcataaaggcgtcaatcgcgataaagagcggcagtcggcgagggtcttttagtttttcttccgccacggcgcgtagaccgggaacaccgtaaaacgggttgctcatattggaaatccaggctttaagcggataaggatagccttcgagcgcggaggtcaacagttcggtaagctggcctgccacaaagggataccacggcgctttggctggataaggggattgcccaccggcaattttgtcgcggtattcttccgatgcttcataagcggttttgctacgggcaatacttaacccggacggtttcacttttccggcaaaactgttcatgttgtagcgggggccgtcgctaacgccgttgaatttgccgccgccgacaaagacgccgccggacaagctgaggttgccgatcagcgcgttaagcatcatgaccgaccaggcgttataaaacccattgccggccatcatgccgccgtgactgatgaccgcagctttacgtccgtgactggtaaaggtttccgccagcgcgataatttgcgcttccggcacgccgcactgttcgctgtattgcgccaacgagagcttttctgccgcctctttcaggcgttgcaacccgctcttcaccgtgacccgttggccgtcggcgagcgtaacgtactgcgtcacgaaaagccgtgcctgtcggcaagtggacgcatcgaccaactcgccgtcggtattcagtacgacaggggtctcttcgccatcgggcgtaagatggcgcagcgtcaggtgttgtccggcaagcgtcggcagctcatccgcaatgaccaggtgcgtggcgttggtccaactttgctcgccggcctgctgcatcgcctgtacgccgggaatcgccagataatcagcattataacgttgattatccatgatccagcggatcatccccattgccagcgccgaatcactgccgggcatgaccggttgccagcgaccgcgaggatcggcgagcaccgttgataaggggagggcgggggcgaccacgacgtattgaaaattctcacgcagtcgggcgctcgccaactgacgtgcctggcgtttaaacggattgccggactgtgccggggaggtgcccataaagagcgcaaactccacgttttcccagtcgggtttgacatgcgggtttttatccagatcgcccatcaatgccccggagccggcccggtaagccagtccacagtaggcgccatgcgcgccgaaattcttgctgccgaagctatttagcgcaaaacgacgcagaaacgcatcgcggccttcgtcgctggtattcgtgaccagtaactgattggttttgggcccgaaactggggtgctttgcgtcaattggcgtatccggcgcatgaatagcgcgcagtccgtccacatgaccttcgccaaacagatcgccgccttccacgacttcttcaataagttgctcaaagctgatgcgctgccatttcccttcgccgcgtttacccacgcgtttcatcggttcaagcagtcgtagcggactgtacaggctttccagcagcgtggcgccgcgcgcgcaggcggttgagcgggcgtcaagaccgctttctcccgccagttgctccatggcttcgctaaaagggacggacgagtcaatcgggtgttcctgcgacaaggggtgatagggattgccggcgatgcgtatcactttgccatcggcattaacccgggcgcggataccgcactgtgtccaacagccgaagcattgcgtcatggcgatggtttgttgtggattttgctgccagtgtgtttgcgcctgcgcctccggaattaacgcattgccaaagatgcggtcgcgcgttaccttgccggacgtcccgtttaacaggccatcaattgcgcgtttcgccacatcacggtagctcagaccaaaagtgaccatcccaccgacggcgagaccgacttttagccactgacgacgggttaaattagccatgttgtaatctcctggtgagtccgttcagcgtttcacgaataataatcagtagcgctatccacaggccgaaggtgccgagaatagccagccagccatccgttccgcctggtaacgagtaagggttaaattgcgcgttgaacttggggacggtttgtacctgaatcaacaatgtccagcgcatcagccaacatagcgccagcgcgctgagaaccagcaggacgcgtcttagctgtgataacggatggcgtagcgccaggctacagaacagcagtgtgcatacccacagcgctacccagccgacagcgtaatatttggctgacagggcgacggtaatccactgacggattgccgtgccggaaagcgtatcgccgctaacccacatggccacaaccagccccagcgccgccagcgtccagatttgtccccacaatatttttggcagccttaccgagtcgcgtcgggcggcgacaatcatcagcgcgaagaacgcctgtaaggcgctaagaaacatcgccacggggaaggcgtagctaaaccagattgggcgcgccagcacaacggagacttcgcggccggtataaatcaacaggcccaccgcgcaaagcgcgctggctaacgccaaccatttagtgacgttgtaacttttattgaataatcgtttaatctgctgcgccaggaaccacagagcgagaaatccggtaaacagcggcaggaataacgctccccagggcatccacgaccagggcgtcggccaggcatagaaatgccagacgcgggcggtctggtgcagatccgccgtcagcgccagcggtgcggtaatcgcacaggtaatggcaatcagtaatgcccgattttcttctgttgcggcgtcttttttccgccagtgaagataacaggcaaacagtgcggcgcaggcggcaatgccaataaaaaagaaatattgtaccgcccacggcagccagctaatgtcctgcgggtgagccagcacttcttcaatgatgagtgaatgcgtcattcagacctcctgccaaagcgcgggctgcgcacggcccattaatggggtgacaaaggcgtcgtccagacccaggtagaaaacatggggcgacgtgccgttttccggctttaataccttgatagcgtcgcgatgctgatgaagcatggtggcgatgcggctatggggatctttgatatcgccaataatacgcgcgccgccgacgcaggactctacgcaagcgggtaacagtccggcttccagacgatggacgcaaaacgtgcatttatcggcagtttgcgtttcatgattgataaatcgggcgtcgtaaggacacgcctggacacaataggcgcagccgacgcagcgtttgttatccaccaccacaatgccatcttcccgctgaaaggtggcttgtaccgggcagaccggcacacagggggggttatcgcaatggttgcacagacgcggcaacagcacattcgtgacttcctgactaccttcacgctggacctggtattggttcaccgtcgtacgaaacgcgccttgcggcgtttggttttcaatagtgcaacttacggtacaggactgacagccgatacaacgccgcagatcgataagcatggcgtaacggtgtcggggagagccttcatgccgctccggcgaaaaaggaaatttcgcttcagccagcggaaccagcgaggcgccagcggtcaggacgccaagctgctggagaaattgccgtttactgctgtccatattgactcccgtccacattgccaacaatgaaacatttgtcacgatgttggttcatgtgtaatgaataaaaaatgtcgatgatttacagtgtaaaaatcgaggcggggtgcgctctattgtggttaaccacatacccggcttgttgttgatctaaaacaacataattgacagggatattggggtgagaggtaaaaccgtaaggcgcctggcggtgttggcggcagtagggctactttgtcatggcgcgtgggcagggacgtggaatatcggtattttggccatgcgcggcgaggcgtctacgcgtagccactggcaaccgttggcaaagacattaagccaacagcttccaggcgaaacctttcacatccagccgctggatctgcatcaaatgcaggaggccgttaaccagggaaccgtgcagtttgtgataaccaacccggcgcaatttgtccaactgaacagccatgcgccgctgcgctggttagcttccctgcgctccacgcgcgatgggaaagcggtgagtaatgttattggcagcgtgattttgacccggcgcgatagcggcatcaccacggcgcatgatctcatcggtaagaccgtcggcgcgattgatgctcaggcgtttggcggctatttattaggctataaagcgctcagcgacgcgggcttacgcccggagcgcgattttcatctccgttttaccggatttcctggcgatgccttagtctatatgctgcgcgaaaaagcggtgcaggcggcaattgtgccagtgtgcctgttagaaaatatggatcaggaaggattgattaataaaaaggactttatcgcgctgctttcccgaccgacgcccctgccttgcttaaccagtacgccgttatatcctgactggtcgttcgcggcgctacctgcggtaagcgatgcgctggcggatcgcgtaacgcgagcgctattcaacgcgcccgccgccgcgtcatttcactggggcgcgcctgcgtccaccagtcaggtggaagccttgctgcgtgatgttcgtcagcaccctcagcagcgtcgactgtggctggatgtcaaaagttggttaatccagcaccagctaatggtcggcggcgtgattctggcgttcttgttgctcacgctcaattatatttgggtcatgctgctggtgcgtcgacgtggaaagcaactggaacgtaatagcgtagttcttcatcagcatgagcgggcgctggaaaccgcccggcaaatgagcgtgttgggtgaaatgacctccgggtttgcccatgagcttaatcagccgctttccgcgattcgacattatgcccaggggtgcctgattcgactgcgcgctgcagatgaacagcatcccttgctgccggcgctggagcagattgaccagcaggcgcaacgcggtgcggatactctgcgtaacctgcgtcactgggtcagccaggcgcagggcaacccggtgctaaccgaagcgtggaaggccatagccattcgcgaggcgattgatcatgtctggcaattgttgcgtatggcgcaacagtttccgacagtgactctgcataccgaggttagcgctgcgctgcgcgtaacgctgccgtcagtgctgctggaacaggtgctggcgaatatcattcttaatgcggctcaggcgggcgccacccatttatggatcgttgctgaacgcactgaaaacggcatcagtattgttttacaggataacgccgggggaatcgatgaggcgctattacgtcaggcgtttcagccgtttatgaccacccgtaaagaggggatgggcttagggctggcgatttgccagcggctggtgcggtatgggcggggcgatatcagcatcaggaaccagaccgcgccggacggtctgtcgggaacggtggttacgatacatttcttacatgaaaatgggggcagggatggcgacaattcatctactggatgatgatacggcggtcactaacgcgtgcgcgtttttactggaaagtctgggatatgacgtaaaatgctggacgcagggggcggattttttggcgcaggccagtctgtatcaggccggggtcgtattactggatatgcgaatgccggtactggatgggcagggcgttcatgatgcgttgcgccagtgcggaagtaccctggcggttgtttttcttaccgggcatggcgatgtaccgatggccgtggagcagatgaaacgcggcgccgtcgattttctgcaaaaaccggtatcggtaaaaccgctacaggcggcgctggagcgtgcgctgacggtttcatcggcagcggtggcgcgtcgtgagattatactgtgttaccagcagttgacgccgaaagagcgtgagctggccagcctggtggcaaaaggatttatgaaccgtgaaattgcggaagcgatgaatatcgcggtgcgtaccgtagaggtgcaccgcgccagagtcatggaaaaaatgcaggccggtagcctggcggaactgattaggcgtttcgaaaaaatggcctcgccagagaccagaatacgaacaacgtatgagccatgaataagagctcgaattctcatgtttgacagcttatcactgatcagtgaattaatggcgatgacgcatcctcacgataatatccgggtaggcgcaatcactttcgtctctactccgttacaaagcgaggctgggtatttcccggcctttctgttatccgaaatccactgaaagcacagcggctggctgaggagataaataataaacgaggggctgtatgcacaaagcatcttctgttgagttaagaacgagtatcgagatggcacatagccttgctcaaattggaatcaggtttgtgccaataccagtagaaacagacgaagaagctagaggtgaatcacgacaaagcgtatcaaaaacgtatggagtagggctctaaactctgtataaaaagtttccagctagctgataacgggaaagaaacagagaagggcacaaatattgtgtactttaatgtgccctttaatttattgattggtggttgaattgtccgtaactttttgatttaagtgcaaatttctaataaattagaacactttcttaaatggtttcactgaaacgtgttcatagactcctgccgctacgtacgggtcagcatcggcccaagcctgagctgcttccagcgactcaaattcagcaataacggttgagccagtaaatcccgcagcc

SEQ ID NO: 48 - DNA, 4395 bp, synthetic construct
  misc_feature 1..4395: note = vector
  source 1..4395: mol_type = other DNA
gacctataaggaaaggccaaacaagaacacggttgcaaaaaccgtgcccttaaatattgaatttctattcagaacactttcttaaattgtcatttggcatattacgaacaattccgcgtaaaaacgttctgttacgctaaacccttatccagcaggctttcaaggatgtaaaccataacactctgcgaactagtgttacattgcgtgtagctttgagtgggcaactttgtgtacacttttgtgtacccaaaaacaaaaatgtgtacccattcaatgatcaccgacacaaagctcaggaaggcgctcggcaagaaaagagatgatatcgagattatttctgattcgcacgggcccatggctaattcccatgtcagccgttaagtgttcctgtgtcactgaaaattgctttgagaggctctaagggcttctcagtgcgttacatccctggcttgttgtccacaaccgttaaaccttaaaagctttaaaagccttatatattcttttttttcttataaaacttaaaaccttagaggctatttaagttgctgatttatattaattttattgttcaaacatgagagcttagtacgtgaaacatgagagcttagtacgttagccatgagagcttagtacgttagccatgagggtttagttcgttaaacatgagagcttagtacgttaaacatgagagcttagtacgtgaaacatgagagcttagtacgtactatcaacaggttgaactgctgatcttcagatcctctacgccggacgcatcgtggccggatcttgcggccgcaaaaattaaaaatgaagttttggaggcctcatttggtgacgaaataactaagcacttgtctcctgtttactcccctgagcttgaggggtcaacatgaaggtcattgatagcaggataataatacagtaaaacgctaaaccaataatccaaatccagccatcccaaattggtagtgaatgattataaataacagtaaacagtaatgggccaataacaccggttgcattggtaaggctcaccaataatccctgtaaagcaccttgctcatgactctttgtttggatagacatcactccctgtaatgcaggtaaagcgatcccaccaccagccaataaaattaaaacagggaaatctaaccaaccttcagatataaacgctaaaaaggcaaatgcactactatctgcaataaattcgagcagtactgccgttttttcgccccatttagtggctattcttcctgccacaaaggcttggaatactgagtgtaaaagaccaagacccgctaatgaaaagccaaccatcatgctattccatccaaaacgattttcggtaaatagcacccacaccgttgcgggaatttggcctatcaattgcgctgaaaaataaataatcaacaaaatgggcatcgttttaaataaagtgatgtacaccgaatttgattgcgtctcaacccctacttcggtatctgtattatcacgtgtatttttggtttcacggaaccaaaacataaccacaaggaaagtgacaatatttagcaacgcagcgataaaaaagggactatgcggtgaaatctctcctgcaaaaccaccaataataggccccgctattaaaccaagcccaaaacttgcccctaaccaaccgaaccacttcacgcgttgagaagctgaggtggtatcggcaatgaccgatgccgcgacagccccagtagctcctgtgatccctgaaagcaaacggcctaaatacagcatccaaagcgcacttgaaaaagccagcaataagtaatccagcgatgcgcctattaatgacaacaacagcactgggcgccgaccaaatcggtcagacatttttccaagccaaggagcaaagataacctgcattaacgcataaagtgcaagcaatacgccaaagtggttagcgatatcttccgaagcaataaattcacgtaataacgttggcaagactggcatgataaggccaatccccatggcatcgagtaacgtaattaccaatgcgatctttgtcgaactattcatttcacttttctctatcactgatagggagtgggaaaataactctatcaatgatagggtgtcaaatcgatggcccccgatggtagtgtggggtctccccatgcgagagtagggaactgccaggcatcaaataaaacgaaaggctcagtcgaaagactgggcctttcgttttatctgttgtttgtcggtgaacgctctcctgagtaggacaaatccgccgggagcggatttgaacgttgcgaagcaacggcccggagggtggcgggcaggacgcccgccataaactgccaggcatcaaattaagcagaaggccatcctgacggatggcctttttgcgtggccagtgccaagcttgcatgcctgcaggtcgactctagaggatccattccggggatccgtcgacctgcagttcgaagttcctattctctagaaagtataggaacttcagagcgcttttgaagctcacgctgccgcaagcactcagggcgcaagggctgctaaaggaagcggaacacgtagaaagccagtccgcagaaacggtgctgaccccggatgaatgtcagctactgggctatctggacaagggaaaacgcaagcgcaaagagaaagcaggtagcttgcagtgggcttacatggcgatagctagactgggcggttttatggacagcaagcgaaccggaattgccagctggggcgccctctggtaaggttgggaagccctgcaaagtaaactggatggctttcttgccgccaaggatctgatggcgcaggggatcaagatctgatcaagagacaggatgaggatcgtttcgcatgattgaacaagatggattgcacgcaggttctccggccgcttgggtggagaggctattcggctatgactgggcacaacagacaatcggctgctctgatgccgccgtgttccggctgtcagcgcaggggcgcccggttctttttgtcaagaccgacctgtccggtgccctgaatgaactgcaggacgaggcagcgcggctatcgtggctggccacgacgggcgttccttgcgcagctgtgctcgacgttgtcactgaagcgggaagggactggctgctattgggcgaagtgccggggcaggatctcctgtcatctcaccttgctcctgccgagaaagtatccatcatggctgatgcaatgcggcggctgcatacgcttgatccggctacctgcccattcgaccaccaagcgaaacatcgcatcgagcgagcacgtactcggatggaagccggtcttgtcgatcaggatgatctggacgaagagcatcaggggctcgcgccagccgaactgttcgccaggctcaaggcgcgcatgcccgacggcgaggatctcgtcgtgacccatggcgatgcctgcttgccgaatatcatggtggaaaatggccgcttttctggattcatcgactgtggccggctgggtgtggcggaccgctatcaggacatagcgttggctacccgtgatattgctgaagagcttggcggcgaatgggctgaccgcttcctcgtgctttacggtatcgccgctcccgattcgcagcgcatcgccttctatcgccttcttgacgagttcttctaataaggggatcttgaagttcctattccgaagttcctattctctagaaagtataggaacttcgaagcagctccagcctacagagctcgaattctcatgtttgacagcttatcactgatcagtgaattaatggcgatgacgcatcctcacgataatatccgggtaggcgcaatcactttcgtctctactccgttacaaagcgaggctgggtatttcccggcctttctgttatccgaaatccactgaaagcacagcggctggctgaggagataaataataaacgaggggctgtatgcacaaagcatcttctgttgagttaagaacgagtatcgagatggcacatagccttgctcaaattggaatcaggtttgtgccaataccagtagaaacagacgaagaagctagaggtgaatcacgacaaagcgtatcaaaaacgtatggagtagggctctaaactctgtataaaaagtttccagctagctgataacgggaaagaaacagagaagggcacaaatattgtgtactttaatgtgccctttaatttattgattggtggttgaattgtccgtaactttttgatttaagtgcaaatttctaataaattagaacactttcttaaatggtttcactgaaacgtgttcatagactcctgccgctacgtacgggtcagcatcggcccaagcctgagctgcttccagcgactcaaattcagcaataacggttgagccagtaaatcccgcagcc

SEQ ID NO: 49 - protein, 28 aa, synthetic construct
  REGION 1..28: note = linker
GSAGSAEAGSNWSHPQFEKGSAGSAAGS

SEQ ID NO: 50 - protein, 12 aa, synthetic construct
  REGION 1..12: note = linker
GSAGSAAGSGEF

SEQ ID NO: 51 - DNA, 84 bp, synthetic construct
  misc_feature 1..84: note = linker
  source 1..84: mol_type = other DNA
ggtagtgctggtagtgctgaagctggtagtaattggagtcatccacaatttgaaaaaggtagtgctggtagtgctgctggtagt

SEQ ID NO: 52 - DNA, 36 bp, synthetic construct
  misc_feature 1..36: note = linker
  source 1..36: mol_type = other DNA
ggtagtgctggtagtgctgctggtagtggtgaattt

SEQ ID NO: 53 - DNA, 3669 bp, Lactobacillus reuteri
  source 1..3669: mol_type = genomic DNA
atgctatcaagaaaaaattataaggaaactatacgaaaacagacacctacaaaacagtactatactattaagaaattaactgttggggttacttcggtattaattggtctatcctttatgggagaactagaaggggatagcgttcatgcggacacgatgacagcaagcagtgagtcaacaagtgttacgtcgacgactgctcaggatggtttaaaaaaatctccacaactctatttgcaagttactgatacaaataacccaagtacaccattaagtgcttcatccacagggactagtaagaatgttacctcatcagctgcggtacaagtgaagtccgctagtgatgaagaagatagtgattctacactagctaagggagaaaataaatttgctcggtcagcagtaaaagattcagtcactgatgggaaaacaagtacagcagaaattaatccggcaaaattaagcagtcctgctttaataacgcaactcaaccaatccttagctaagagcagtacgagtgatgcagcaaaagctaatgatgagttagaaattaaagcaacagatccgactaattatccaaactgtggcgatgtgtatgggccattatttgaattggatgctagcggacagcttgttaataaagatgaagttatatctcttaaagatatgtatattttccaaatattgaaattagtaaatacaaaagatagtgactttcaatatgtaatattaacaatgaatcgtaaagatactgcagataggtctgtatatctttttgtaactggaagcaattatagtaatgctgttgttgttaaagtaaagccaaatgatacttatgaattaagtaaaactggatatagtgttacttatacagaaccaacaactataaatggacattatgttgatggaactttttatgttacaggaagtacttacgatgatggttttataatgccagattggcaactgcagcaccttcagattatatatagtttaggaaattatgatccaagcaatactgacgcaacatcagtttgtgaaataatgccaagttatgaaaaggtaccggtaattaaatatagtggagtaccttcaaatattagccaacctaaggtttacattaccgggtttacgggtcaagagtttaacgttacagatattattaacaattataagaaagtttttaagggctactatcttcaaaatcctaatgtggcgtccatgggaactctttcccaatttgagaatggtggttattacttaaagacatattatgataatgatggtaatgttgactttaagggcttgtatcatcaaattgatgatcagggaacaatgagtgtgagtgttcttaatgcagataataaaacaattgttggacctgaaaatattcttgctggtaaatcgcataactttaactttaatggtcataactggattgcgcggaatccttatgtcactagttcagctcacgaagtcatattaaagtatgctaagttaggttcagttattcctgttgatgaaaacggaaataaaataaacgatggatggcaatatgttaatgatccagatgatgcttccaaagccactagcccatatgaaaaagcgccagttatcgatggttatgtagctgtaaatccagatgaaacgatcgttcttcctcataacttaagtagtgacacaaagatttattaccgaaagaggattaaagttacctatagtggtagtgacagcaagacctacgatggtaacccagctaacttcgagccaacgacagttcagtggagtggcttgaaaggactgaacacttcaaccttaacgtccgctgacttcacgtggaatactgcggataagaaggcaccaacggatgccggtaagtacacacttagtttgaatacgaccggagaagcagccttacgtaaggctaacccgaactatgatctcaagacaattagcggtagttacacctacacgattaatccactagggattgataaagttacctatagtggtagtgacagcaagacctacgatggtaacccagctaacttcgagccaacgacagttcagtggagtggcttgaaaggactgaacacttcaaccttaacgtccgctgacttcacgtggaatactgcggataagaaggcaccaacggatgccggtaagtacacacttagtttgaatacgaccggagaagcagccttacgtaaggctaacccgaactatgatctcaagacaattagcggtagttacacctacacgattaatccactagggattgataaagttacctatagtggtagtgacagcaagacctacgatggtaacccagctaacttcgagccaacgacagttcagtggagtggcttgaaaggactgaacacttcaaccttaacgtccgctgacttcacgtggaatactgcggataagaaggcaccaacggatgccggtaagtacacacttagtttgaatacgaccggagaagcagccttacgtaaggctaacccgaactatgatctcaagacaattagcggtagttacacctacacgattaatccactagggattgataaagttacctatagtggtagtgacagcaagacctacgatggtaacccagctaacttcgagccaacgacagttcagtggagtggcttgaaaggactgaacacttcaaccttaacgtccgctgacttcacgtggaatactgcggataagaaggcaccaacggatgccggtaagtacacacttagtttgaatacgaccggagaagcagccttacgtaaggctaacccgaactatgatctcaagacaattagcggtagttacacctacacgattaatccactagggattgataaagttacctatagtggtagtgacagcaagacctacgatggtaacccagctaacttcgagccaacgacagttcagtggagtggcttgaaaggactgaacacttcaaccttaacgtccgctgacttcacgtggaatactgcggataagaaggcaccaacggatgccggtaagtacacacttagtttgaatacgaccggagaagcagccttacgtaaggctaacccgaactatgatctcaagacaattagcggtagttacacctacacgattaatccactagggattgtgactgtaaattacaagggctatgataagaaagtctatgatggtcaacctggaacgattaatccgggtaaattaacgtggagtaagttgccagatggtacttcattgaagatgccaacatggagtatagatgatttcgcttgggaaacagctgatggcttagcaccaacggcagtaggaacttatcggattatcttgacggatgctggtaaggctgcactaaagaagattaatccaaattatgacttaagcagtattactggtgtctttacttatgaaattaagccagcacagacaccagaaatcttaggccaaacacctgagcaacaaccaggccaaaatactaatcaatcaggagctgaaaacggctttggttcttctacaaggcctaatgcatcaactaactccaatcttaatcaacttccacagactggtaatgagcattctaatactgcacttgctggtctagcattggctttcttgactgctatgcttggtttgggcaagaagcgtaaacatgattag

SEQ ID NO: 54 - DNA, 18 bp, synthetic construct
  misc_feature 1..18: note = Primer
  source 1..18: mol_type = other DNA
cggctaccacccaaggaa

SEQ ID NO: 55 - DNA, 18 bp, synthetic construct
  misc_feature 1..18: note = Primer
  source 1..18: mol_type = other DNA
gctggaattaccgcggct

SEQ ID NO: 56 - DNA, 21 bp, synthetic construct
  misc_feature 1..21: note = Primer
  source 1..21: mol_type = other DNA
accgtgaatcttggctgtaac

SEQ ID NO: 57 - DNA, 21 bp, synthetic construct
  misc_feature 1..21: note = Primer
  source 1..21: mol_type = other DNA
gcagcaaatcgcttgggatta

SEQ ID NO: 58 - DNA, 20 bp, synthetic construct
  misc_feature 1..20: note = Primer
  source 1..20: mol_type = other DNA
tgtcagtcatcgcccatgtg

SEQ ID NO: 59 - DNA, 21 bp, synthetic construct
  misc_feature 1..21: note = Primer
  source 1..21: mol_type = other DNA
catccttgcgagtgtcagtga

SEQ ID NO: 60 - DNA, 24 bp, synthetic construct
  misc_feature 1..24: note = Primer
  source 1..24: mol_type = other DNA
catcttctcaaaattcgagtgaca

SEQ ID NO: 61 - DNA, 23 bp, synthetic construct
  misc_feature 1..23: note = Primer
  source 1..23: mol_type = other DNA
tgggagtagacaaggtacaaccc

SEQ ID NO: 62 - DNA, 23 bp, synthetic construct
  misc_feature 1..23: note = Primer
  source 1..23: mol_type = other DNA
tcaagtggcatagatgtggaaga

SEQ ID NO: 63 - DNA, 21 bp, synthetic construct
  misc_feature 1..21: note = Primer
  source 1..21: mol_type = other DNA
tggctctgcaggattttcatg

SEQ ID NO: 64 - DNA, 20 bp, synthetic construct
  misc_feature 1..20: note = Primer
  source 1..20: mol_type = other DNA
agggccctttgctatggtgt

SEQ ID NO: 65 - DNA, 20 bp, synthetic construct
  misc_feature 1..20: note = Primer
  source 1..20: mol_type = other DNA
tggccacagttttcagggat

SEQ ID NO: 66 - DNA, 20 bp, synthetic construct
  misc_feature 1..20: note = Primer
  source 1..20: mol_type = other DNA
agcttccttgtgcaagtgtc

SEQ ID NO: 67 - DNA, 20 bp, synthetic construct
  misc_feature 1..20: note = Primer
  source 1..20: mol_type = other DNA
cccttcatcttttggggtcc

SEQ ID NO: 68 - DNA, 20 bp, synthetic construct
  misc_feature 1..20: note = Primer
  source 1..20: mol_type = other DNA
tccctctgtgatctgggaag

SEQ ID NO: 69 - DNA, 20 bp, synthetic construct
  misc_feature 1..20: note = Primer
  source 1..20: mol_type = other DNA
ctcgaccctgaaagtgaagg

SEQ ID NO: 70 - DNA, 22 bp, synthetic construct
  misc_feature 1..22: note = Primer
  source 1..22: mol_type = other DNA
cccgtataaccatcaccatcat

SEQ ID NO: 71 - DNA, 21 bp, synthetic construct
  misc_feature 1..21: note = Primer
  source 1..21: mol_type = other DNA
ggcatctttcttggcaacttc

SEQ ID NO: 72 - DNA, 17 bp, synthetic construct
  misc_feature 1..17: note = Primer
  source 1..17: mol_type = other DNA
gccagatcccgaaacca

SEQ ID NO: 73 - DNA, 20 bp, synthetic construct
  misc_feature 1..20: note = Primer
  source 1..20: mol_type = other DNA
tataggagtctcggcagtca

SEQ ID NO: 74 - protein, 5 aa, synthetic construct
LPXTG

SEQ ID NO: 75 - protein, 12 aa, synthetic construct
YSIRKXXXGXXS